European Patent Application EP 4 566 619 A1, published June 11, 2025. Title: Targeting modules against CD19 and CD20 for use in a method for stimulating a reversed chimeric antigen receptor-mediated immune response in a mammal. Applicant: AvenCell Europe GmbH. Application EP. The sequence listing filed with the application follows.

SEQUENCE LISTING (137 sequences)

SEQ ID NO: 1 - protein, 260 aa, synthetic construct
  source 1..260: note = CD19-binding scFv
DIQLTQSPASLAVSLGQRATISCKASQSVDYDGDSYLNWYQQIPGQPPKLLIYDASNLVSGIPPRFSGSGSGTDFTLNIHPVEKVDAATYHCQQSTEDPWTFGGGTKLEIKGGGGSGGGGSGGGGSGGGGSGGGGSQVQLQQSGAELVRPGSSVKISCKASGYAFSSYWMNWVKQRPGQGLEWIGQIWPGDGDTNYNGKFKGKATLTADESSSTAYMQLSSLASEDSAVYFCARRETTTVGRYYYAMDYWGQGTTVTVSS

SEQ ID NO: 2 - protein, 260 aa, synthetic construct
  source 1..260: note = CD19-binding scFv
QVQLQQSGAELVRPGSSVKISCKASGYAFSSYWMNWVKQRPGQGLEWIGQIWPGDGDTNYNGKFKGKATLTADESSSTAYMQLSSLASEDSAVYFCARRETTTVGRYYYAMDYWGQGTTVTVSSGGGGSGGGGSGGGGSGGGGSGGGGSDIQLTQSPASLAVSLGQRATISCKASQSVDYDGDSYLNWYQQIPGQPPKLLIYDASNLVSGIPPRFSGSGSGTDFTLNIHPVEKVDAATYHCQQSTEDPWTFGGGTKLEIK

SEQ ID NO: 3 - protein, 116 aa, synthetic construct
  source 1..116: note = CD19-binding VHH
EVQLVESGGGLVQPGGSLRLSCAASGFSFSDFWMSWVRQAPGKGLEWVATISQAGSEKDYVDSVKGRFTISRDNAKKSLYLQMNSLRAEDTAVYYCASGVYSFDYRGQGTLVTVSS

SEQ ID NO: 4 - protein, 121 aa, Lama glama
  VARIANT 5: note = Xaa can be any naturally occurring amino acid
  VARIANT 14: note = Xaa can be any naturally occurring amino acid
  VARIANT 43: note = Xaa can be any naturally occurring amino acid
  VARIANT 44: note = Xaa can be any naturally occurring amino acid
  VARIANT 45: note = Xaa can be any naturally occurring amino acid
  VARIANT 62: note = Xaa can be any naturally occurring amino acid
  VARIANT 65: note = Xaa can be any naturally occurring amino acid
  VARIANT 75: note = Xaa can be any naturally occurring amino acid
  VARIANT 76: note = Xaa can be any naturally occurring amino acid
  VARIANT 79: note = Xaa can be any naturally occurring amino acid
  VARIANT 87: note = Xaa can be any naturally occurring amino acid
  VARIANT 88: note = Xaa can be any naturally occurring amino acid
  VARIANT 116: note = Xaa can be any naturally occurring amino acid
QVQLXESGGGLVQXGGSLRLSCAASGRTFSNYNMGWFRQAPGXXXEFVAAIDWSGGSPYYAXSVXGRFTISRDNXXNTXYLQMNSLXXEDTAVYYCAAPLSYGSTWLADYWGQGTXVTVSS

SEQ ID NO: 5 - protein, 121 aa, Lama glama
QVQLQESGGGLVQAGGSLRLSCAASGRTFSNYNMGWFRQAPGKEREFVAAIDWSGGSPYYAASVRGRFTISRDNAENTVYLQMNSLKPEDTAVYYCAAPLSYGSTWLADYWGQGTQVTVSS

SEQ ID NO: 6 - protein, 121 aa, synthetic construct
  source 1..121: note = CD20-binding VHH
QVQLVESGGGLVQPGGSLRLSCAASGRTFSNYNMGWFRQAPGQGLEFVAAIDWSGGSPYYADSVKGRFTISRDNSKNTLYLQMNSLRAEDTAVYYCAAPLSYGSTWLADYWGQGTLVTVSS

SEQ ID NO: 7 - protein, 121 aa, synthetic construct
  source 1..121: note = CD20-binding VHH
QVQLVESGGGLVQPGGSLRLSCAASGRTFSNYNMGWFRQAPGQGLEFVAAIDWSGGSPYYAASVRGRFTISRDNSKNTLYLQMNSLRAEDTAVYYCAAPLSYGSTWLADYWGQGTLVTVSS

SEQ ID NO: 8 - protein, 15 aa, Mus musculus
KASQSVDYDGDSYLN

SEQ ID NO: 9 - protein, 7 aa, Mus musculus
DASNLVS

SEQ ID NO: 10 - protein, 9 aa, Mus musculus
QQSTEDPWT

SEQ ID NO: 11 - protein, 7 aa, Mus musculus
GYAFSSY

SEQ ID NO: 12 - protein, 6 aa, Mus musculus
WPGDGD

SEQ ID NO: 13 - protein, 59 aa, Mus musculus
DGDTNYNGKFKGKATLTADESSSTAYMQLSSLASEDSAVYFCARRETTTVGRYYYAMDY

SEQ ID NO: 14 - protein, 10 aa, Lama glama
GRTFSNYNMG

SEQ ID NO: 15 - protein, 17 aa, synthetic construct
  source 1..17: note = CD20-binding CDR
AIDWSGGSPYYADSVKG

SEQ ID NO: 16 - protein, 12 aa, Lama glama
PLSYGSTWLADY

SEQ ID NO: 17 - protein, 17 aa, synthetic construct
  source 1..17: note = CD20-binding CDR
AIDWSGGSPYYAASVRG

SEQ ID NO: 18 - protein, 33 aa, Saccharomyces cerevisiae
RMKQLEPKVEELLPKNYHLENEVARLKKLVGER

SEQ ID NO: 19 - protein, 14 aa, Saccharomyces cerevisiae
NYHLENEVARLKKL

SEQ ID NO: 20 - protein, 51 aa, Homo sapiens
MDPDLEIRAAFLRQRNTALRTEVAELEQEVQRLENEVSQYETRYGPLGGGK

SEQ ID NO: 21 - protein, 51 aa, Homo sapiens
MDPDLEIEAAFLERENTALETRVAELRQRVQRLRNRVSQYRTRYGPLGGGK

SEQ ID NO: 22 - protein, 10 aa, Homo sapiens
KPLPEVTDEY

SEQ ID NO: 23 - protein, 20 aa, Homo sapiens
  VARIANT 16: note = Xaa can be alanine or serine
LEKEALKKIIEDQQEXLNKW

SEQ ID NO: 24 - protein, 20 aa, Homo sapiens
LEKEALKKIIEDQQEALNKW

SEQ ID NO: 25 - protein, 5 aa, synthetic construct
  source 1..5: note = linker sequence
GGGGS

SEQ ID NO: 26 - protein, 25 aa, synthetic construct
  source 1..25: note = linker sequence
GGGGSGGGGSGASAAGGGGSGGGGS

SEQ ID NO: 27 - protein, 25 aa, synthetic construct
  source 1..25: note = linker sequence
GGGGSGGGGSGGGGSGGGGSGGGGS

SEQ ID NO: 28 - protein, 8 aa, synthetic construct
  source 1..8: note = 5B9-binding CDR
GYTFTHYY

SEQ ID NO: 29 - protein, 8 aa, synthetic construct
  source 1..8: note = 5B9-binding CDR
VNPSNGGT

SEQ ID NO: 30 - protein, 13 aa, synthetic construct
  source 1..13: note = 5B9-binding CDR
ARSEYDYGLGFAY

SEQ ID NO: 31 - protein, 12 aa, synthetic construct
  source 1..12: note = 5B9-binding CDR
QSLLNSRTPKNY

SEQ ID NO: 32 - protein, 8 aa, synthetic construct
  source 1..8: note = 5B9-binding CDR
KQSYNLLT

SEQ ID NO: 33 - protein, 113 aa, synthetic construct
  source 1..113: note = La-epitope-binding VL
  VARIANT 24: note = Xaa can be any naturally occurring amino acid
  VARIANT 35: note = Xaa can be any naturally occurring amino acid
  VARIANT 61: note = Xaa can be any naturally occurring amino acid
  VARIANT 101: note = Xaa can be any naturally occurring amino acid
DIVMTQSPDSLAVSLGERATINCXSSQSLLNSRTXKNYLAWYQQKPGQPPKLLIYWASTRXSGVPDRFSGSGSGTDFTLTISSLQAEDVAVYYCKQSYNLXTFGGGTKVEILK

SEQ ID NO: 34 - protein, 112 aa, synthetic construct
  source 1..112: note = 5B9-binding VL
DIVMTQSPDSLAVSLGERATINCKSSQSLLNSRTPKNYLAWYQQKPGQPPKLLIYWASTRKSGVPDRFSGSGSGTDFTLTISSLQAEDVAVYYCKQSYNLLTFGGGTKVEIK

SEQ ID NO: 35 - protein, 120 aa, synthetic construct
  source 1..120: note = 5B9-binding VH
QVQLVQSGAEVKKPGASVKVSCKASGYTFTHYYIYWVRQAPGQGLEWMGGVNPSNGGTHFNEKFKSRVTMTRDTSISTAYMELSRLRSDDTAVYYCARSEYDYGLGFAYWGQGTLVTVSS

SEQ ID NO: 36 - protein, 112 aa, synthetic construct
  source 1..112: note = 7B6-binding VL
DIVMTQSPDSLAVSLGERATINCRSSQSLLDSRTKKNYLAWYQQKPGQPPKLLIYWASTRESGVPDRFSGSGSGTDFTLTISSLQAEDVAVYYCKQSYNLPTFGGGTKVEIK

SEQ ID NO: 37 - protein, 118 aa, synthetic construct
  source 1..118: note = 7B6-binding VH
EVQLVESGGGLVQPGGSLRLSCAASGFTFSDFWMNWVRQAPGKGLEWVGQIRNKPNNYETYYSDSLKGRFTISRDDSKSITYLQMNSLRAEDTAVYYCTLGNSWFAYWGQGTLVTVSS

SEQ ID NO: 38 - protein, 219 aa, synthetic construct
  source 1..219: note = humanized Fab fragment
GQVQLVQSGAEVKKPGASVKVSCKASGYTFTHYYIYWVRQAPGQGLEWMGGVNPSNGGTHFNEKFKSRVTMTRDTSISTAYMELSRLRSDDTAVYYCARSEYDYGLGFAYWGQGTLVTVSSASTKGPSVFPLAPSSKSTSGGTAALGCLVKDYFPEPVTVSWNSGALTSGVHTFPAVLQSSGLYSLSSVVTVPSSSLGTQTYICNVNHKPSNTKVDKKV

SEQ ID NO: 39 - protein, 219 aa, synthetic construct
  source 1..219: note = humanized Fab fragment
DIVMTQSPDSLAVSLGERATINCKSSQSLLNSRTPKNYLAWYQQKPGQPPKLLIYWASTRKSGVPDRFSGSGSGTDFTLTISSLQAEDVAVYYCKQSYNLLTFGGGTKVEIKRTVAAPSVFIFPPSDEQLKSGTASVVCLLNNFYPREAKVQWKVDNALQSGNSQESVTEQDSKDSTYSLSSTLTLSKADYEKHKVYACEVTHQGLSSPVTKSFNRGEC

SEQ ID NO: 40 - protein, 231 aa, synthetic construct
  source 1..231: note = silenced IgG1 Fc-Knob
EPKSCDKTHTCPPCPAPPVAGPSVFLFPPKPKDTLMISRTPEVTCVVVDVSHEDPEVKFNWYVDGVEVHNAKTKPREEQYNSTYRVVSVLTVLHQDWLNGKEYKCKVSNKGLPSSIEKTISKAKGQPREPQVYTLPPSRDELTKNQVSLWCLVKGFYPSDIAVEWESNGQPENNYKTTPPVLDSDGSFFLYSKLTVDKSRWQQGNVFSCSVMHEALHNHYTQKSLSLSPGK

SEQ ID NO: 41 - protein, 231 aa, synthetic construct
  source 1..231: note = silenced IgG1 Fc-Hole
EPKSCDKTHTCPPCPAPPVAGPSVFLFPPKPKDTLMISRTPEVTCVVVDVSHEDPEVKFNWYVDGVEVHNAKTKPREEQYNSTYRVVSVLTVLHQDWLNGKEYKCKVSNKGLPSSIEKTISKAKGQPREPQVYTLPPSRDELTKNQVSLSCAVKGFYPSDIAVEWESNGQPENNYKTTPPVLDSDGSFFLVSKLTVDKSRWQQGNVFSCSVMHEALHNHYTQKSLSLSPGK

SEQ ID NO: 42 - protein, 22 aa, Homo sapiens
MDMRAPAQVFGFLLLWFPGARC

SEQ ID NO: 43 - protein, 19 aa, Mus musculus
MGWSCIILFLVATATGVHS

SEQ ID NO: 44 - protein, 450 aa, synthetic construct
  source 1..450: note = targeting module chain
GQVQLVQSGAEVKKPGASVKVSCKASGYTFTHYYIYWVRQAPGQGLEWMGGVNPSNGGTHFNEKFKSRVTMTRDTSISTAYMELSRLRSDDTAVYYCARSEYDYGLGFAYWGQGTLVTVSSASTKGPSVFPLAPSSKSTSGGTAALGCLVKDYFPEPVTVSWNSGALTSGVHTFPAVLQSSGLYSLSSVVTVPSSSLGTQTYICNVNHKPSNTKVDKKVEPKSCDKTHTCPPCPAPPVAGPSVFLFPPKPKDTLMISRTPEVTCVVVDVSHEDPEVKFNWYVDGVEVHNAKTKPREEQYNSTYRVVSVLTVLHQDWLNGKEYKCKVSNKGLPSSIEKTISKAKGQPREPQVYTLPPSRDELTKNQVSLWCLVKGFYPSDIAVEWESNGQPENNYKTTPPVLDSDGSFFLYSKLTVDKSRWQQGNVFSCSVMHEALHNHYTQKSLSLSPGK

SEQ ID NO: 45 - protein, 469 aa, synthetic construct
  source 1..469: note = targeting module chain
MGWSCIILFLVATATGVHSGQVQLVQSGAEVKKPGASVKVSCKASGYTFTHYYIYWVRQAPGQGLEWMGGVNPSNGGTHFNEKFKSRVTMTRDTSISTAYMELSRLRSDDTAVYYCARSEYDYGLGFAYWGQGTLVTVSSASTKGPSVFPLAPSSKSTSGGTAALGCLVKDYFPEPVTVSWNSGALTSGVHTFPAVLQSSGLYSLSSVVTVPSSSLGTQTYICNVNHKPSNTKVDKKVEPKSCDKTHTCPPCPAPPVAGPSVFLFPPKPKDTLMISRTPEVTCVVVDVSHEDPEVKFNWYVDGVEVHNAKTKPREEQYNSTYRVVSVLTVLHQDWLNGKEYKCKVSNKGLPSSIEKTISKAKGQPREPQVYTLPPSRDELTKNQVSLWCLVKGFYPSDIAVEWESNGQPENNYKTTPPVLDSDGSFFLYSKLTVDKSRWQQGNVFSCSVMHEALHNHYTQKSLSLSPGK

SEQ ID NO: 46 - protein, 350 aa, synthetic construct
  source 1..350: note = targeting module chain
DIVMTQSPDSLAVSLGERATINCKSSQSLLNSRTPKNYLAWYQQKPGQPPKLLIYWASTRKSGVPDRFSGSGSGTDFTLTISSLQAEDVAVYYCKQSYNLLTFGGGTKVEIKRTVAAPSVFIFPPSDEQLKSGTASVVCLLNNFYPREAKVQWKVDNALQSGNSQESVTEQDSKDSTYSLSSTLTLSKADYEKHKVYACEVTHQGLSSPVTKSFNRGECGGGGSGGGGSGGGGSEVQLVESGGGLVQPGGSLRLSCAASGFSFSDFWMSWVRQAPGKGLEWVATISQAGSEKDYVDSVKGRFTISRDNAKKSLYLQMNSLRAEDTAVYYCASGVYSFDYRGQGTLVTVSS

SEQ ID NO: 47 - protein, 372 aa, synthetic construct
  source 1..372: note = targeting module chain
MDMRAPAQVFGFLLLWFPGARCDIVMTQSPDSLAVSLGERATINCKSSQSLLNSRTPKNYLAWYQQKPGQPPKLLIYWASTRKSGVPDRFSGSGSGTDFTLTISSLQAEDVAVYYCKQSYNLLTFGGGTKVEIKRTVAAPSVFIFPPSDEQLKSGTASVVCLLNNFYPREAKVQWKVDNALQSGNSQESVTEQDSKDSTYSLSSTLTLSKADYEKHKVYACEVTHQGLSSPVTKSFNRGECGGGGSGGGGSGGGGSEVQLVESGGGLVQPGGSLRLSCAASGFSFSDFWMSWVRQAPGKGLEWVATISQAGSEKDYVDSVKGRFTISRDNAKKSLYLQMNSLRAEDTAVYYCASGVYSFDYRGQGTLVTVSS

SEQ ID NO: 48 - protein, 353 aa, synthetic construct
  source 1..353: note = targeting module chain
GQVQLQESGGGLVQAGGSLRLSCAASGRTFSNYNMGWFRQAPGKEREFVAAIDWSGGSPYYAASVRGRFTISRDNAENTVYLQMNSLKPEDTAVYYCAAPLSYGSTWLADYWGQGTQVTVSSEPKSCDKTHTCPPCPAPPVAGPSVFLFPPKPKDTLMISRTPEVTCVVVDVSHEDPEVKFNWYVDGVEVHNAKTKPREEQYNSTYRVVSVLTVLHQDWLNGKEYKCKVSNKGLPSSIEKTISKAKGQPREPQVYTLPPSRDELTKNQVSLSCAVKGFYPSDIAVEWESNGQPENNYKTTPPVLDSDGSFFLVSKLTVDKSRWQQGNVFSCSVMHEALHNHYTQKSLSLSPGK

SEQ ID NO: 49 - protein, 372 aa, synthetic construct
  source 1..372: note = targeting module chain
MGWSCIILFLVATATGVHSGQVQLQESGGGLVQAGGSLRLSCAASGRTFSNYNMGWFRQAPGKEREFVAAIDWSGGSPYYAASVRGRFTISRDNAENTVYLQMNSLKPEDTAVYYCAAPLSYGSTWLADYWGQGTQVTVSSEPKSCDKTHTCPPCPAPPVAGPSVFLFPPKPKDTLMISRTPEVTCVVVDVSHEDPEVKFNWYVDGVEVHNAKTKPREEQYNSTYRVVSVLTVLHQDWLNGKEYKCKVSNKGLPSSIEKTISKAKGQPREPQVYTLPPSRDELTKNQVSLSCAVKGFYPSDIAVEWESNGQPENNYKTTPPVLDSDGSFFLVSKLTVDKSRWQQGNVFSCSVMHEALHNHYTQKSLSLSPGK

SEQ ID NO: 50 - protein, 353 aa, synthetic construct
  source 1..353: note = targeting module chain
GQVQLVESGGGLVQPGGSLRLSCAASGRTFSNYNMGWFRQAPGQGLEFVAAIDWSGGSPYYADSVKGRFTISRDNSKNTLYLQMNSLRAEDTAVYYCAAPLSYGSTWLADYWGQGTLVTVSSEPKSCDKTHTCPPCPAPPVAGPSVFLFPPKPKDTLMISRTPEVTCVVVDVSHEDPEVKFNWYVDGVEVHNAKTKPREEQYNSTYRVVSVLTVLHQDWLNGKEYKCKVSNKGLPSSIEKTISKAKGQPREPQVYTLPPSRDELTKNQVSLSCAVKGFYPSDIAVEWESNGQPENNYKTTPPVLDSDGSFFLVSKLTVDKSRWQQGNVFSCSVMHEALHNHYTQKSLSLSPGK

SEQ ID NO: 51 - protein, 372 aa, synthetic construct
  source 1..372: note = targeting module chain
MGWSCIILFLVATATGVHSGQVQLVESGGGLVQPGGSLRLSCAASGRTFSNYNMGWFRQAPGQGLEFVAAIDWSGGSPYYADSVKGRFTISRDNSKNTLYLQMNSLRAEDTAVYYCAAPLSYGSTWLADYWGQGTLVTVSSEPKSCDKTHTCPPCPAPPVAGPSVFLFPPKPKDTLMISRTPEVTCVVVDVSHEDPEVKFNWYVDGVEVHNAKTKPREEQYNSTYRVVSVLTVLHQDWLNGKEYKCKVSNKGLPSSIEKTISKAKGQPREPQVYTLPPSRDELTKNQVSLSCAVKGFYPSDIAVEWESNGQPENNYKTTPPVLDSDGSFFLVSKLTVDKSRWQQGNVFSCSVMHEALHNHYTQKSLSLSPGK

SEQ ID NO: 52 - protein, 353 aa, synthetic construct
  source 1..353: note = targeting module chain
GQVQLVESGGGLVQPGGSLRLSCAASGRTFSNYNMGWFRQAPGQGLEFVAAIDWSGGSPYYAASVRGRFTISRDNSKNTLYLQMNSLRAEDTAVYYCAAPLSYGSTWLADYWGQGTLVTVSSEPKSCDKTHTCPPCPAPPVAGPSVFLFPPKPKDTLMISRTPEVTCVVVDVSHEDPEVKFNWYVDGVEVHNAKTKPREEQYNSTYRVVSVLTVLHQDWLNGKEYKCKVSNKGLPSSIEKTISKAKGQPREPQVYTLPPSRDELTKNQVSLSCAVKGFYPSDIAVEWESNGQPENNYKTTPPVLDSDGSFFLVSKLTVDKSRWQQGNVFSCSVMHEALHNHYTQKSLSLSPGK

SEQ ID NO: 53 - protein, 372 aa, synthetic construct
  source 1..372: note = targeting module chain
MGWSCIILFLVATATGVHSGQVQLVESGGGLVQPGGSLRLSCAASGRTFSNYNMGWFRQAPGQGLEFVAAIDWSGGSPYYAASVRGRFTISRDNSKNTLYLQMNSLRAEDTAVYYCAAPLSYGSTWLADYWGQGTLVTVSSEPKSCDKTHTCPPCPAPPVAGPSVFLFPPKPKDTLMISRTPEVTCVVVDVSHEDPEVKFNWYVDGVEVHNAKTKPREEQYNSTYRVVSVLTVLHQDWLNGKEYKCKVSNKGLPSSIEKTISKAKGQPREPQVYTLPPSRDELTKNQVSLSCAVKGFYPSDIAVEWESNGQPENNYKTTPPVLDSDGSFFLVSKLTVDKSRWQQGNVFSCSVMHEALHNHYTQKSLSLSPGK

SEQ ID NO: 54 - protein, 484 aa, synthetic construct
  source 1..484: note = targeting module chain
GQVQLQESGGGLVQAGGSLRLSCAASGRTFSNYNMGWFRQAPGKEREFVAAIDWSGGSPYYAASVRGRFTISRDNAENTVYLQMNSLKPEDTAVYYCAAPLSYGSTWLADYWGQGTQVTVSSGGGGSGGGGSQVQLQESGGGLVQAGGSLRLSCAASGRTFSNYNMGWFRQAPGKEREFVAAIDWSGGSPYYAASVRGRFTISRDNAENTVYLQMNSLKPEDTAVYYCAAPLSYGSTWLADYWGQGTQVTVSSEPKSCDKTHTCPPCPAPPVAGPSVFLFPPKPKDTLMISRTPEVTCVVVDVSHEDPEVKFNWYVDGVEVHNAKTKPREEQYNSTYRVVSVLTVLHQDWLNGKEYKCKVSNKGLPSSIEKTISKAKGQPREPQVYTLPPSRDELTKNQVSLSCAVKGFYPSDIAVEWESNGQPENNYKTTPPVLDSDGSFFLVSKLTVDKSRWQQGNVFSCSVMHEALHNHYTQKSLSLSPGK

SEQ ID NO: 55 - protein, 503 aa, synthetic construct
  source 1..503: note = targeting module chain
MGWSCIILFLVATATGVHSGQVQLQESGGGLVQAGGSLRLSCAASGRTFSNYNMGWFRQAPGKEREFVAAIDWSGGSPYYAASVRGRFTISRDNAENTVYLQMNSLKPEDTAVYYCAAPLSYGSTWLADYWGQGTQVTVSSGGGGSGGGGSQVQLQESGGGLVQAGGSLRLSCAASGRTFSNYNMGWFRQAPGKEREFVAAIDWSGGSPYYAASVRGRFTISRDNAENTVYLQMNSLKPEDTAVYYCAAPLSYGSTWLADYWGQGTQVTVSSEPKSCDKTHTCPPCPAPPVAGPSVFLFPPKPKDTLMISRTPEVTCVVVDVSHEDPEVKFNWYVDGVEVHNAKTKPREEQYNSTYRVVSVLTVLHQDWLNGKEYKCKVSNKGLPSSIEKTISKAKGQPREPQVYTLPPSRDELTKNQVSLSCAVKGFYPSDIAVEWESNGQPENNYKTTPPVLDSDGSFFLVSKLTVDKSRWQQGNVFSCSVMHEALHNHYTQKSLSLSPGK

SEQ ID NO: 56 - protein, 484 aa, synthetic construct
  source 1..484: note = targeting module chain
GQVQLVESGGGLVQPGGSLRLSCAASGRTFSNYNMGWFRQAPGQGLEFVAAIDWSGGSPYYADSVKGRFTISRDNSKNTLYLQMNSLRAEDTAVYYCAAPLSYGSTWLADYWGQGTLVTVSSGGGGSGGGGSQVQLVESGGGLVQPGGSLRLSCAASGRTFSNYNMGWFRQAPGQGLEFVAAIDWSGGSPYYADSVKGRFTISRDNSKNTLYLQMNSLRAEDTAVYYCAAPLSYGSTWLADYWGQGTLVTVSSEPKSCDKTHTCPPCPAPPVAGPSVFLFPPKPKDTLMISRTPEVTCVVVDVSHEDPEVKFNWYVDGVEVHNAKTKPREEQYNSTYRVVSVLTVLHQDWLNGKEYKCKVSNKGLPSSIEKTISKAKGQPREPQVYTLPPSRDELTKNQVSLSCAVKGFYPSDIAVEWESNGQPENNYKTTPPVLDSDGSFFLVSKLTVDKSRWQQGNVFSCSVMHEALHNHYTQKSLSLSPGK

SEQ ID NO: 57 - protein, 503 aa, synthetic construct
  source 1..503: note = targeting module chain
MGWSCIILFLVATATGVHSGQVQLVESGGGLVQPGGSLRLSCAASGRTFSNYNMGWFRQAPGQGLEFVAAIDWSGGSPYYADSVKGRFTISRDNSKNTLYLQMNSLRAEDTAVYYCAAPLSYGSTWLADYWGQGTLVTVSSGGGGSGGGGSQVQLVESGGGLVQPGGSLRLSCAASGRTFSNYNMGWFRQAPGQGLEFVAAIDWSGGSPYYADSVKGRFTISRDNSKNTLYLQMNSLRAEDTAVYYCAAPLSYGSTWLADYWGQGTLVTVSSEPKSCDKTHTCPPCPAPPVAGPSVFLFPPKPKDTLMISRTPEVTCVVVDVSHEDPEVKFNWYVDGVEVHNAKTKPREEQYNSTYRVVSVLTVLHQDWLNGKEYKCKVSNKGLPSSIEKTISKAKGQPREPQVYTLPPSRDELTKNQVSLSCAVKGFYPSDIAVEWESNGQPENNYKTTPPVLDSDGSFFLVSKLTVDKSRWQQGNVFSCSVMHEALHNHYTQKSLSLSPGK

SEQ ID NO: 58 - protein, 484 aa, synthetic construct
  source 1..484: note = targeting module chain
GQVQLVESGGGLVQPGGSLRLSCAASGRTFSNYNMGWFRQAPGQGLEFVAAIDWSGGSPYYAASVRGRFTISRDNSKNTLYLQMNSLRAEDTAVYYCAAPLSYGSTWLADYWGQGTLVTVSSGGGGSGGGGSQVQLVESGGGLVQPGGSLRLSCAASGRTFSNYNMGWFRQAPGQGLEFVAAIDWSGGSPYYAASVRGRFTISRDNSKNTLYLQMNSLRAEDTAVYYCAAPLSYGSTWLADYWGQGTLVTVSSEPKSCDKTHTCPPCPAPPVAGPSVFLFPPKPKDTLMISRTPEVTCVVVDVSHEDPEVKFNWYVDGVEVHNAKTKPREEQYNSTYRVVSVLTVLHQDWLNGKEYKCKVSNKGLPSSIEKTISKAKGQPREPQVYTLPPSRDELTKNQVSLSCAVKGFYPSDIAVEWESNGQPENNYKTTPPVLDSDGSFFLVSKLTVDKSRWQQGNVFSCSVMHEALHNHYTQKSLSLSPGK

SEQ ID NO: 59 - protein, 503 aa, synthetic construct
  source 1..503: note = targeting module chain
MGWSCIILFLVATATGVHSGQVQLVESGGGLVQPGGSLRLSCAASGRTFSNYNMGWFRQAPGQGLEFVAAIDWSGGSPYYAASVRGRFTISRDNSKNTLYLQMNSLRAEDTAVYYCAAPLSYGSTWLADYWGQGTLVTVSSGGGGSGGGGSQVQLVESGGGLVQPGGSLRLSCAASGRTFSNYNMGWFRQAPGQGLEFVAAIDWSGGSPYYAASVRGRFTISRDNSKNTLYLQMNSLRAEDTAVYYCAAPLSYGSTWLADYWGQGTLVTVSSEPKSCDKTHTCPPCPAPPVAGPSVFLFPPKPKDTLMISRTPEVTCVVVDVSHEDPEVKFNWYVDGVEVHNAKTKPREEQYNSTYRVVSVLTVLHQDWLNGKEYKCKVSNKGLPSSIEKTISKAKGQPREPQVYTLPPSRDELTKNQVSLSCAVKGFYPSDIAVEWESNGQPENNYKTTPPVLDSDGSFFLVSKLTVDKSRWQQGNVFSCSVMHEALHNHYTQKSLSLSPGK

SEQ ID NO: 60 - protein, 484 aa, synthetic construct
  source 1..484: note = targeting module chain
GQVQLQESGGGLVQAGGSLRLSCAASGRTFSNYNMGWFRQAPGKEREFVAAIDWSGGSPYYAASVRGRFTISRDNAENTVYLQMNSLKPEDTAVYYCAAPLSYGSTWLADYWGQGTQVTVSSGGGGSGGGGSGGGGSEVQLVESGGGLVQPGGSLRLSCAASGFSFSDFWMSWVRQAPGKGLEWVATISQAGSEKDYVDSVKGRFTISRDNAKKSLYLQMNSLRAEDTAVYYCASGVYSFDYRGQGTLVTVSSEPKSCDKTHTCPPCPAPPVAGPSVFLFPPKPKDTLMISRTPEVTCVVVDVSHEDPEVKFNWYVDGVEVHNAKTKPREEQYNSTYRVVSVLTVLHQDWLNGKEYKCKVSNKGLPSSIEKTISKAKGQPREPQVYTLPPSRDELTKNQVSLSCAVKGFYPSDIAVEWESNGQPENNYKTTPPVLDSDGSFFLVSKLTVDKSRWQQGNVFSCSVMHEALHNHYTQKSLSLSPGK

SEQ ID NO: 61 - protein, 503 aa, synthetic construct
  source 1..503: note = targeting module chain
MGWSCIILFLVATATGVHSGQVQLQESGGGLVQAGGSLRLSCAASGRTFSNYNMGWFRQAPGKEREFVAAIDWSGGSPYYAASVRGRFTISRDNAENTVYLQMNSLKPEDTAVYYCAAPLSYGSTWLADYWGQGTQVTVSSGGGGSGGGGSGGGGSEVQLVESGGGLVQPGGSLRLSCAASGFSFSDFWMSWVRQAPGKGLEWVATISQAGSEKDYVDSVKGRFTISRDNAKKSLYLQMNSLRAEDTAVYYCASGVYSFDYRGQGTLVTVSSEPKSCDKTHTCPPCPAPPVAGPSVFLFPPKPKDTLMISRTPEVTCVVVDVSHEDPEVKFNWYVDGVEVHNAKTKPREEQYNSTYRVVSVLTVLHQDWLNGKEYKCKVSNKGLPSSIEKTISKAKGQPREPQVYTLPPSRDELTKNQVSLSCAVKGFYPSDIAVEWESNGQPENNYKTTPPVLDSDGSFFLVSKLTVDKSRWQQGNVFSCSVMHEALHNHYTQKSLSLSPGK

SEQ ID NO: 62 - protein, 484 aa, synthetic construct
  source 1..484: note = targeting module chain
GQVQLVESGGGLVQPGGSLRLSCAASGRTFSNYNMGWFRQAPGQGLEFVAAIDWSGGSPYYADSVKGRFTISRDNSKNTLYLQMNSLRAEDTAVYYCAAPLSYGSTWLADYWGQGTLVTVSSGGGGSGGGGSGGGGSEVQLVESGGGLVQPGGSLRLSCAASGFSFSDFWMSWVRQAPGKGLEWVATISQAGSEKDYVDSVKGRFTISRDNAKKSLYLQMNSLRAEDTAVYYCASGVYSFDYRGQGTLVTVSSEPKSCDKTHTCPPCPAPPVAGPSVFLFPPKPKDTLMISRTPEVTCVVVDVSHEDPEVKFNWYVDGVEVHNAKTKPREEQYNSTYRVVSVLTVLHQDWLNGKEYKCKVSNKGLPSSIEKTISKAKGQPREPQVYTLPPSRDELTKNQVSLSCAVKGFYPSDIAVEWESNGQPENNYKTTPPVLDSDGSFFLVSKLTVDKSRWQQGNVFSCSVMHEALHNHYTQKSLSLSPGK

SEQ ID NO: 63 - protein, 503 aa, synthetic construct
  source 1..503: note = targeting module chain
MGWSCIILFLVATATGVHSGQVQLVESGGGLVQPGGSLRLSCAASGRTFSNYNMGWFRQAPGQGLEFVAAIDWSGGSPYYADSVKGRFTISRDNSKNTLYLQMNSLRAEDTAVYYCAAPLSYGSTWLADYWGQGTLVTVSSGGGGSGGGGSGGGGSEVQLVESGGGLVQPGGSLRLSCAASGFSFSDFWMSWVRQAPGKGLEWVATISQAGSEKDYVDSVKGRFTISRDNAKKSLYLQMNSLRAEDTAVYYCASGVYSFDYRGQGTLVTVSSEPKSCDKTHTCPPCPAPPVAGPSVFLFPPKPKDTLMISRTPEVTCVVVDVSHEDPEVKFNWYVDGVEVHNAKTKPREEQYNSTYRVVSVLTVLHQDWLNGKEYKCKVSNKGLPSSIEKTISKAKGQPREPQVYTLPPSRDELTKNQVSLSCAVKGFYPSDIAVEWESNGQPENNYKTTPPVLDSDGSFFLVSKLTVDKSRWQQGNVFSCSVMHEALHNHYTQKSLSLSPGK

SEQ ID NO: 64 - protein, 484 aa, synthetic construct
  source 1..484: note = targeting module chain
GQVQLVESGGGLVQPGGSLRLSCAASGRTFSNYNMGWFRQAPGQGLEFVAAIDWSGGSPYYAASVRGRFTISRDNSKNTLYLQMNSLRAEDTAVYYCAAPLSYGSTWLADYWGQGTLVTVSSGGGGSGGGGSGGGGSEVQLVESGGGLVQPGGSLRLSCAASGFSFSDFWMSWVRQAPGKGLEWVATISQAGSEKDYVDSVKGRFTISRDNAKKSLYLQMNSLRAEDTAVYYCASGVYSFDYRGQGTLVTVSSEPKSCDKTHTCPPCPAPPVAGPSVFLFPPKPKDTLMISRTPEVTCVVVDVSHEDPEVKFNWYVDGVEVHNAKTKPREEQYNSTYRVVSVLTVLHQDWLNGKEYKCKVSNKGLPSSIEKTISKAKGQPREPQVYTLPPSRDELTKNQVSLSCAVKGFYPSDIAVEWESNGQPENNYKTTPPVLDSDGSFFLVSKLTVDKSRWQQGNVFSCSVMHEALHNHYTQKSLSLSPGK

SEQ ID NO: 65 - protein, 503 aa, synthetic construct
  source 1..503: note = targeting module chain
MGWSCIILFLVATATGVHSGQVQLVESGGGLVQPGGSLRLSCAASGRTFSNYNMGWFRQAPGQGLEFVAAIDWSGGSPYYAASVRGRFTISRDNSKNTLYLQMNSLRAEDTAVYYCAAPLSYGSTWLADYWGQGTLVTVSSGGGGSGGGGSGGGGSEVQLVESGGGLVQPGGSLRLSCAASGFSFSDFWMSWVRQAPGKGLEWVATISQAGSEKDYVDSVKGRFTISRDNAKKSLYLQMNSLRAEDTAVYYCASGVYSFDYRGQGTLVTVSSEPKSCDKTHTCPPCPAPPVAGPSVFLFPPKPKDTLMISRTPEVTCVVVDVSHEDPEVKFNWYVDGVEVHNAKTKPREEQYNSTYRVVSVLTVLHQDWLNGKEYKCKVSNKGLPSSIEKTISKAKGQPREPQVYTLPPSRDELTKNQVSLSCAVKGFYPSDIAVEWESNGQPENNYKTTPPVLDSDGSFFLVSKLTVDKSRWQQGNVFSCSVMHEALHNHYTQKSLSLSPGK

SEQ ID NO: 66 - protein, 483 aa, synthetic construct
  source 1..483: note = targeting module chain
EVQLVESGGGLVQPGGSLRLSCAASGFSFSDFWMSWVRQAPGKGLEWVATISQAGSEKDYVDSVKGRFTISRDNAKKSLYLQMNSLRAEDTAVYYCASGVYSFDYRGQGTLVTVSSEPKSCDKTHTCPPCPAPPVAGPSVFLFPPKPKDTLMISRTPEVTCVVVDVSHEDPEVKFNWYVDGVEVHNAKTKPREEQYNSTYRVVSVLTVLHQDWLNGKEYKCKVSNKGLPSSIEKTISKAKGQPREPQVYTLPPSRDELTKNQVSLSCAVKGFYPSDIAVEWESNGQPENNYKTTPPVLDSDGSFFLVSKLTVDKSRWQQGNVFSCSVMHEALHNHYTQKSLSLSPGKGGGGSGGGGSGGGGSQVQLQESGGGLVQAGGSLRLSCAASGRTFSNYNMGWFRQAPGKEREFVAAIDWSGGSPYYAASVRGRFTISRDNAENTVYLQMNSLKPEDTAVYYCAAPLSYGSTWLADYWGQGTQVTVSS

SEQ ID NO: 67 - protein, 502 aa, synthetic construct
  source 1..502: note = targeting module chain
MGWSCIILFLVATATGVHSEVQLVESGGGLVQPGGSLRLSCAASGFSFSDFWMSWVRQAPGKGLEWVATISQAGSEKDYVDSVKGRFTISRDNAKKSLYLQMNSLRAEDTAVYYCASGVYSFDYRGQGTLVTVSSEPKSCDKTHTCPPCPAPPVAGPSVFLFPPKPKDTLMISRTPEVTCVVVDVSHEDPEVKFNWYVDGVEVHNAKTKPREEQYNSTYRVVSVLTVLHQDWLNGKEYKCKVSNKGLPSSIEKTISKAKGQPREPQVYTLPPSRDELTKNQVSLSCAVKGFYPSDIAVEWESNGQPENNYKTTPPVLDSDGSFFLVSKLTVDKSRWQQGNVFSCSVMHEALHNHYTQKSLSLSPGKGGGGSGGGGSGGGGSQVQLQESGGGLVQAGGSLRLSCAASGRTFSNYNMGWFRQAPGKEREFVAAIDWSGGSPYYAASVRGRFTISRDNAENTVYLQMNSLKPEDTAVYYCAAPLSYGSTWLADYWGQGTQVTVSS

SEQ ID NO: 68 - protein, 483 aa, synthetic construct
  source 1..483: note = targeting module chain
EVQLVESGGGLVQPGGSLRLSCAASGFSFSDFWMSWVRQAPGKGLEWVATISQAGSEKDYVDSVKGRFTISRDNAKKSLYLQMNSLRAEDTAVYYCASGVYSFDYRGQGTLVTVSSEPKSCDKTHTCPPCPAPPVAGPSVFLFPPKPKDTLMISRTPEVTCVVVDVSHEDPEVKFNWYVDGVEVHNAKTKPREEQYNSTYRVVSVLTVLHQDWLNGKEYKCKVSNKGLPSSIEKTISKAKGQPREPQVYTLPPSRDELTKNQVSLSCAVKGFYPSDIAVEWESNGQPENNYKTTPPVLDSDGSFFLVSKLTVDKSRWQQGNVFSCSVMHEALHNHYTQKSLSLSPGKGGGGSGGGGSGGGGSQVQLVESGGGLVQPGGSLRLSCAASGRTFSNYNMGWFRQAPGQGLEFVAAIDWSGGSPYYADSVKGRFTISRDNSKNTLYLQMNSLRAEDTAVYYCAAPLSYGSTWLADYWGQGTLVTVSS

SEQ ID NO: 69 - protein, 502 aa, synthetic construct
  source 1..502: note = targeting module chain
MGWSCIILFLVATATGVHSEVQLVESGGGLVQPGGSLRLSCAASGFSFSDFWMSWVRQAPGKGLEWVATISQAGSEKDYVDSVKGRFTISRDNAKKSLYLQMNSLRAEDTAVYYCASGVYSFDYRGQGTLVTVSSEPKSCDKTHTCPPCPAPPVAGPSVFLFPPKPKDTLMISRTPEVTCVVVDVSHEDPEVKFNWYVDGVEVHNAKTKPREEQYNSTYRVVSVLTVLHQDWLNGKEYKCKVSNKGLPSSIEKTISKAKGQPREPQVYTLPPSRDELTKNQVSLSCAVKGFYPSDIAVEWESNGQPENNYKTTPPVLDSDGSFFLVSKLTVDKSRWQQGNVFSCSVMHEALHNHYTQKSLSLSPGKGGGGSGGGGSGGGGSQVQLVESGGGLVQPGGSLRLSCAASGRTFSNYNMGWFRQAPGQGLEFVAAIDWSGGSPYYADSVKGRFTISRDNSKNTLYLQMNSLRAEDTAVYYCAAPLSYGSTWLADYWGQGTLVTVSS

SEQ ID NO: 70 - protein, 483 aa, synthetic construct
  source 1..483: note = targeting module chain
EVQLVESGGGLVQPGGSLRLSCAASGFSFSDFWMSWVRQAPGKGLEWVATISQAGSEKDYVDSVKGRFTISRDNAKKSLYLQMNSLRAEDTAVYYCASGVYSFDYRGQGTLVTVSSEPKSCDKTHTCPPCPAPPVAGPSVFLFPPKPKDTLMISRTPEVTCVVVDVSHEDPEVKFNWYVDGVEVHNAKTKPREEQYNSTYRVVSVLTVLHQDWLNGKEYKCKVSNKGLPSSIEKTISKAKGQPREPQVYTLPPSRDELTKNQVSLSCAVKGFYPSDIAVEWESNGQPENNYKTTPPVLDSDGSFFLVSKLTVDKSRWQQGNVFSCSVMHEALHNHYTQKSLSLSPGKGGGGSGGGGSGGGGSQVQLVESGGGLVQPGGSLRLSCAASGRTFSNYNMGWFRQAPGQGLEFVAAIDWSGGSPYYAASVRGRFTISRDNSKNTLYLQMNSLRAEDTAVYYCAAPLSYGSTWLADYWGQGTLVTVSS

SEQ ID NO: 71 - protein, 502 aa, synthetic construct
  source 1..502: note = targeting module chain
MGWSCIILFLVATATGVHSEVQLVESGGGLVQPGGSLRLSCAASGFSFSDFWMSWVRQAPGKGLEWVATISQAGSEKDYVDSVKGRFTISRDNAKKSLYLQMNSLRAEDTAVYYCASGVYSFDYRGQGTLVTVSSEPKSCDKTHTCPPCPAPPVAGPSVFLFPPKPKDTLMISRTPEVTCVVVDVSHEDPEVKFNWYVDGVEVHNAKTKPREEQYNSTYRVVSVLTVLHQDWLNGKEYKCKVSNKGLPSSIEKTISKAKGQPREPQVYTLPPSRDELTKNQVSLSCAVKGFYPSDIAVEWESNGQPENNYKTTPPVLDSDGSFFLVSKLTVDKSRWQQGNVFSCSVMHEALHNHYTQKSLSLSPGKGGGGSGGGGSGGGGSQVQLVESGGGLVQPGGSLRLSCAASGRTFSNYNMGWFRQAPGQGLEFVAAIDWSGGSPYYAASVRGRFTISRDNSKNTLYLQMNSLRAEDTAVYYCAAPLSYGSTWLADYWGQGTLVTVSS

SEQ ID NO: 72 - protein, 484 aa, synthetic construct
  source 1..484: note = targeting module chain
DIQLTQSPASLAVSLGQRATISCKASQSVDYDGDSYLNWYQQIPGQPPKLLIYDASNLVSGIPPRFSGSGSGTDFTLNIHPVEKVDAATYHCQQSTEDPWTFGGGTKLEIKGGGGSGGGGSGGGGSGGGGSGGGGSQVQLQQSGAELVRPGSSVKISCKASGYAFSSYWMNWVKQRPGQGLEWIGQIWPGDGDTNYNGKFKGKATLTADESSSTAYMQLSSLASEDSAVYFCARRETTTVGRYYYAMDYWGQGTTVTVSSGGGGSDIVMTQSPDSLAVSLGERATINCKSSQSLLNSRTPKNYLAWYQQKPGQPPKLLIYWASTRKSGVPDRFSGSGSGTDFTLTISSLQAEDVAVYYCKQSYNLLTFGGGTKVEIKRTVAAPSVFIFPPSDEQLKSGTASVVCLLNNFYPREAKVQWKVDNALQSGNSQESVTEQDSKDSTYSLSSTLTLSKADYEKHKVYACEVTHQGLSSPVTKSFNRGEC

SEQ ID NO: 73 - protein, 506 aa, synthetic construct
  source 1..506: note = targeting module chain
MDMRAPAQVFGFLLLWFPGARCDIQLTQSPASLAVSLGQRATISCKASQSVDYDGDSYLNWYQQIPGQPPKLLIYDASNLVSGIPPRFSGSGSGTDFTLNIHPVEKVDAATYHCQQSTEDPWTFGGGTKLEIKGGGGSGGGGSGGGGSGGGGSGGGGSQVQLQQSGAELVRPGSSVKISCKASGYAFSSYWMNWVKQRPGQGLEWIGQIWPGDGDTNYNGKFKGKATLTADESSSTAYMQLSSLASEDSAVYFCARRETTTVGRYYYAMDYWGQGTTVTVSSGGGGSDIVMTQSPDSLAVSLGERATINCKSSQSLLNSRTPKNYLAWYQQKPGQPPKLLIYWASTRKSGVPDRFSGSGSGTDFTLTISSLQAEDVAVYYCKQSYNLLTFGGGTKVEIKRTVAAPSVFIFPPSDEQLKSGTASVVCLLNNFYPREAKVQWKVDNALQSGNSQESVTEQDSKDSTYSLSSTLTLSKADYEKHKVYACEVTHQGLSSPVTKSFNRGEC

SEQ ID NO: 74 - protein, 485 aa, synthetic construct
  source 1..485: note = targeting module chain
GQVQLQQSGAELVRPGSSVKISCKASGYAFSSYWMNWVKQRPGQGLEWIGQIWPGDGDTNYNGKFKGKATLTADESSSTAYMQLSSLASEDSAVYFCARRETTTVGRYYYAMDYWGQGTTVTVSSGGGGSGGGGSGGGGSGGGGSGGGGSDIQLTQSPASLAVSLGQRATISCKASQSVDYDGDSYLNWYQQIPGQPPKLLIYDASNLVSGIPPRFSGSGSGTDFTLNIHPVEKVDAATYHCQQSTEDPWTFGGGTKLEIKGGGGSDIVMTQSPDSLAVSLGERATINCKSSQSLLNSRTPKNYLAWYQQKPGQPPKLLIYWASTRKSGVPDRFSGSGSGTDFTLTISSLQAEDVAVYYCKQSYNLLTFGGGTKVEIKRTVAAPSVFIFPPSDEQLKSGTASVVCLLNNFYPREAKVQWKVDNALQSGNSQESVTEQDSKDSTYSLSSTLTLSKADYEKHKVYACEVTHQGLSSPVTKSFNRGEC

SEQ ID NO: 75 - protein, 504 aa, synthetic construct
  source 1..504: note = targeting module chain
MGWSCIILFLVATATGVHSGQVQLQQSGAELVRPGSSVKISCKASGYAFSSYWMNWVKQRPGQGLEWIGQIWPGDGDTNYNGKFKGKATLTADESSSTAYMQLSSLASEDSAVYFCARRETTTVGRYYYAMDYWGQGTTVTVSSGGGGSGGGGSGGGGSGGGGSGGGGSDIQLTQSPASLAVSLGQRATISCKASQSVDYDGDSYLNWYQQIPGQPPKLLIYDASNLVSGIPPRFSGSGSGTDFTLNIHPVEKVDAATYHCQQSTEDPWTFGGGTKLEIKGGGGSDIVMTQSPDSLAVSLGERATINCKSSQSLLNSRTPKNYLAWYQQKPGQPPKLLIYWASTRKSGVPDRFSGSGSGTDFTLTISSLQAEDVAVYYCKQSYNLLTFGGGTKVEIKRTVAAPSVFIFPPSDEQLKSGTASVVCLLNNFYPREAKVQWKVDNALQSGNSQESVTEQDSKDSTYSLSSTLTLSKADYEKHKVYACEVTHQGLSSPVTKSFNRGEC

SEQ ID NO: 76 - protein, 241 aa, synthetic construct
  source 1..241: note = targeting module chain
MDMRAPAQVFGFLLLWFPGARCDIVMTQSPDSLAVSLGERATINCKSSQSLLNSRTPKNYLAWYQQKPGQPPKLLIYWASTRKSGVPDRFSGSGSGTDFTLTISSLQAEDVAVYYCKQSYNLLTFGGGTKVEIKRTVAAPSVFIFPPSDEQLKSGTASVVCLLNNFYPREAKVQWKVDNALQSGNSQESVTEQDSKDSTYSLSSTLTLSKADYEKHKVYACEVTHQGLSSPVTKSFNRGEC

SEQ ID NO: 77 - protein, 347 aa, synthetic construct
  source 1..347: note = switchable chimeric antigen receptor
EFKPLPEVTDEYAAAGPGGGGSKILVKQSPMLVAYDNAVNLSCKYSYNLFSREFRASLHKGLDSAVEVCVVYGNYSQQLQVYSKTGFNCDGKLGNESVTFYLQNLYVNQTDIYFCKIEVMAPPPALDNEKSNGTIIHVKGKHLCPSPLFPGPSKPFWVLVVVGGVLACYSLLVTVAFIIFWVRSKRSRGGHSDYMNMTPRRPGPTRKHYQPYAPPRDFAAYRSGGGGSGGGASGGGGSFSRSADAPAYQQGQNQLYNELNLGRREEYDVLDKRRGRDPEMGGKPRRKNPQEGLYNELQKDKMAEAYSEIGMKGERRRGKGHDGLYQGLSTATKDTYGALHMQALPPR

SEQ ID NO: 78 - protein, 220 aa, synthetic construct
  source 1..220: note = switchable chimeric antigen receptor
EFKPLPEVTDEYAAAGGSGGSESKYGPPCPPCPTRGLDFACDIYIWAPLAGTCGVLLLSLVITLYCKRGRKKLLYIFKQPFMRPVQTTQEEDGCSCRFPEEEEGGCELRVKFSRSADAPAYKQGQNQLYNELNLGRREEYDVLDKRRGRDPEMGGKPRRKNPQEGLYNELQKDKMAEAYSEIGMKGERRRGKGHDGLYQGLSTATKDTYDALHMQALPPR

SEQ ID NO: 79 - protein, 244 aa, synthetic construct
  source 1..244: note = switchable chimeric antigen receptor
EFKPLPEVTDEYAAAGGSGGSTTTPAPRPPTPAPTIASQPLSLRPEACRPAAGGAVHTRGLDFACDIYIWAPLAGTCGVLLLSLVITLYCKRGRKKLLYIFKQPFMRPVQTTQEEDGCSCRFPEEEEGGCELRVKFSRSADAPAYKQGQNQLYNELNLGRREEYDVLDKRRGRDPEMGGKPRRKNPQEGLYNELQKDKMAEAYSEIGMKGERRRGKGHDGLYQGLSTATKDTYDALHMQALPPR

SEQ ID NO: 80 - protein, 240 aa, synthetic construct
  source 1..240: note = switchable chimeric antigen receptor
EFKPLPEVTDEYAAAGGSGGSIEVMYPPPYLDNEKSNGTIIHVKGKHLCPSPLFPGPSKPFWVLVVVGGVLACYSLLVTVAFIIFWVRSKRSRLLHSDYMNMTPRRPGPTRKHYQPYAPPRDFAAYRSRVKFSRSADAPAYQQGQNQLYNELNLGRREEYDVLDKRRGRDPEMGGKPRRKNPQEGLYNELQKDKMAEAYSEIGMKGERRRGKGHDGLYQGLSTATKDTYDALHMQALPPR

SEQ ID NO: 81 - protein, 257 aa, synthetic construct
  source 1..257: note = switchable chimeric antigen receptor
EFKPLPEVTDEYAAAGGSGGSFVPVFLPAKPTTTPAPRPPTPAPTIASQPLSLRPEACRPAAGGAVHTRGLDFACDIYIWAPLAGTCGVLLLSLVITLYCNHRNRSKRSRLLHSDYMNMTPRRPGPTRKHYQPYAPPRDFAAYRSRVKFSRSADAPAYQQGQNQLYNELNLGRREEYDVLDKRRGRDPEMGGKPRRKNPQEGLYNELQKDKMAEAYSEIGMKGERRRGKGHDGLYQGLSTATKDTYDALHMQALPPR

SEQ ID NO: 82 - protein, 239 aa, synthetic construct
  source 1..239: note = switchable chimeric antigen receptor
EFKPLPEVTDEYGGSGGSGGSKPLPEVTDEYAAAGGSGGSESKYGPPCPPCPTRGLDFACDIYIWAPLAGTCGVLLLSLVITLYCKRGRKKLLYIFKQPFMRPVQTTQEEDGCSCRFPEEEEGGCELRVKFSRSADAPAYKQGQNQLYNELNLGRREEYDVLDKRRGRDPEMGGKPRRKNPQEGLYNELQKDKMAEAYSEIGMKGERRRGKGHDGLYQGLSTATKDTYDALHMQALPPR

SEQ ID NO: 83 - protein, 258 aa, synthetic construct
  source 1..258: note = switchable chimeric antigen receptor
EFKPLPEVTDEYGGSGGSGGSKPLPEVTDEYGGSGGSGGSKPLPEVTDEYAAAGGSGGSESKYGPPCPPCPTRGLDFACDIYIWAPLAGTCGVLLLSLVITLYCKRGRKKLLYIFKQPFMRPVQTTQEEDGCSCRFPEEEEGGCELRVKFSRSADAPAYKQGQNQLYNELNLGRREEYDVLDKRRGRDPEMGGKPRRKNPQEGLYNELQKDKMAEAYSEIGMKGERRRGKGHDGLYQGLSTATKDTYDALHMQALPPR

SEQ ID NO: 84 - protein, 347 aa, synthetic construct
  source 1..347: note = switchable chimeric antigen receptor
EFKPLPEVTDEYAAAGPGGGGSKILVKQSPMLVAYDNAVNLSCKYSYNLFSREFRASLHKGLDSAVEVCVVYGNYSQQLQVYSKTGFNCDGKLGNESVTFYLQNLYVNQTDIYFCKIEVMAPPPALDNEKSNGTIIHVKGKHLCPSPLFPGPSKPFWVLVVVGGVLACYSLLVTVAFIIFWVRSRRSRGGHSDYMNMTPRRPGPTRKHYQPYAPPRDFAAYRSGGGGSGGGASGGGGSFSRSADAPAYQQGQNQLYNELNLGRREEYDVLDRRRGRDPEMGGRPRRRNPQEGLYNELQRDRMAEAYSEIGMRGERRRGRGHDGLYQGLSTATRDTYGALHMQALPPR

SEQ ID NO: 85 - protein, 349 aa, synthetic construct
  source 1..349: note = switchable chimeric antigen receptor
EFSKPLPEVTDEYKNAAAGGSGGSKILVKQSPMLVAYDNAVNLSCKYSYNLFSREFRASLHKGLDSAVEVCVVYGNYSQQLQVYSKTGFNCDGKLGNESVTFYLQNLYVNQTDIYFCKIEVMAPPPALDNEKSNGTIIHVKGKHLCPSPLFPGPSKPFWVLVVVGGVLACYSLLVTVAFIIFWVRSKRSRGGHSDYMNMTPRRPGPTRKHYQPYAPPRDFAAYRSGGGGSGGGASGGGGSFSRSADAPAYQQGQNQLYNELNLGRREEYDVLDKRRGRDPEMGGKPRRKNPQEGLYNELQKDKMAEAYSEIGMKGERRRGKGHDGLYQGLSTATKDTYGALHMQALPPR

SEQ ID NO: 86 - protein, 203 aa, synthetic construct
  source 1..203: note = switchable chimeric antigen receptor
EFKPLPEVTDEYESKYGPPCPPCPDIYIWAPLAGTCGVLLLSLVITLYCKRGRKKLLYIFKQPFMRPVQTTQEEDGCSCRFPEEEEGGCELRVKFSRSADAPAYQQGQNQLYNELNLGRREEYDVLDKRRGRDPEMGGKPRRKNPQEGLYNELQKDKMAEAYSEIGMKGERRRGKGHDGLYQGLSTATKDTYDALHMQALPPR

SEQ ID NO: 87 - protein, 206 aa, synthetic construct
  source 1..206: note = switchable chimeric antigen receptor
EFKPLPEVTDEYAAAESKYGPPCPPCPDIYIWAPLAGTCGVLLLSLVITLYCKRGRKKLLYIFKQPFMRPVQTTQEEDGCSCRFPEEEEGGCELRVKFSRSADAPAYQQGQNQLYNELNLGRREEYDVLDKRRGRDPEMGGKPRRKNPQEGLYNELQKDKMAEAYSEIGMKGERRRGKGHDGLYQGLSTATKDTYDALHMQALPPR

SEQ ID NO: 88 - protein, 212 aa, synthetic construct
  source 1..212: note = switchable chimeric antigen receptor
EFKPLPEVTDEYAAAGGSGGSESKYGPPCPPCPDIYIWAPLAGTCGVLLLSLVITLYCKRGRKKLLYIFKQPFMRPVQTTQEEDGCSCRFPEEEEGGCELRVKFSRSADAPAYQQGQNQLYNELNLGRREEYDVLDKRRGRDPEMGGKPRRKNPQEGLYNELQKDKMAEAYSEIGMKGERRRGKGHDGLYQGLSTATKDTYDALHMQALPPR

SEQ ID NO: 89 - protein, 207 aa, synthetic construct
  source 1..207: note = switchable chimeric antigen receptor
SKPLPEVTDEYKNAAAESKYGPPCPPCPDIYIWAPLAGTCGVLLLSLVITLYCKRGRKKLLYIFKQPFMRPVQTTQEEDGCSCRFPEEEEGGCELRVKFSRSADAPAYQQGQNQLYNELNLGRREEYDVLDKRRGRDPEMGGKPRRKNPQEGLYNELQKDKMAEAYSEIGMKGERRRGKGHDGLYQGLSTATKDTYDALHMQALPPR

SEQ ID NO: 90 - protein, 373 aa, synthetic construct
  source 1..373: note = switchable chimeric antigen receptor
ENGDNEKMAALEAKICHQIEYYFGDFNLPRDKFLKEQIKLDEGWVPLEIMIKFNRLNRLTTDFNVIVEALSKSKAELMEISEDKTKIRRSPSKPLPEVTDEYKNDVKNRSVYIKGFPTDATLDDIKEWLEDKGQVLNIQMRRTLHKAFKGSIFVVFDSIESAKKFVETPGQKYKETDLLILFESKYGPPCPPCPDIYIWAPLAGTCGVLLLSLVITLYCKRGRKKLLYIFKQPFMRPVQTTQEEDGCSCRFPEEEEGGCELRVKFSRSADAPAYQQGQNQLYNELNLGRREEYDVLDKRRGRDPEMGGKPRRKNPQEGLYNELQKDKMAEAYSEIGMKGERRRGKGHDGLYQGLSTATKDTYDALHMQALPPR

SEQ ID NO: 91 - protein, 220 aa, synthetic construct
  source 1..220: note = switchable chimeric antigen receptor
EFKPLPEVTDEYGGGGSEFKPLPEVTDEYESKYGPPCPPCPDIYIWAPLAGTCGVLLLSLVITLYCKRGRKKLLYIFKQPFMRPVQTTQEEDGCSCRFPEEEEGGCELRVKFSRSADAPAYQQGQNQLYNELNLGRREEYDVLDKRRGRDPEMGGKPRRKNPQEGLYNELQKDKMAEAYSEIGMKGERRRGKGHDGLYQGLSTATKDTYDALHMQALPPR

SEQ ID NO: 92 - protein, 208 aa, synthetic construct
  source 1..208: note = switchable chimeric antigen receptor
EFKPLPEVTDEYAAAESKYGPPCPPCPMFWVLVVVGGVLACYSLLVTVAFIIFWVRSKRSRLLHSDYMNMTPRRPGPTRKHYQPYAPPRDFAAYRSRVKFSRSADAPAYQQGQNQLYNELNLGRREEYDVLDKRRGRDPEMGGKPRRKNPQEGLYNELQKDKMAEAYSEIGMKGERRRGKGHDGLYQGLSTATKDTYDALHMQALPPR

SEQ ID NO: 93 - protein, 209 aa, synthetic construct
  source 1..209: note = switchable chimeric antigen receptor
EFKPLPEVTDEYAAAESKYGPPCPPCPMFWVLVVVGGVLACYSLLVTVAFIIFWVKRGRKKLLYIFKQPFMRPVQTTQEEDGCSCRFPEEEEGGCELRVKFSRSADAPAYQQGQNQLYNELNLGRREEYDVLDKRRGRDPEMGGKPRRKNPQEGLYNELQKDKMAEAYSEIGMKGERRRGKGHDGLYQGLSTATKDTYDALHMQALPPR

SEQ ID NO: 94 - protein, 222 aa, synthetic construct
  source 1..222: note = switchable chimeric antigen receptor
EFKPLPEVTDEYGGGGSEFKPLPEVTDEYESKYGPPCPPCPMFWVLVVVGGVLACYSLLVTVAFIIFWVRSKRSRLLHSDYMNMTPRRPGPTRKHYQPYAPPRDFAAYRSRVKFSRSADAPAYQQGQNQLYNELNLGRREEYDVLDKRRGRDPEMGGKPRRKNPQEGLYNELQKDKMAEAYSEIGMKGERRRGKGHDGLYQGLSTATKDTYDALHMQALPPR

SEQ ID NO: 95 - protein, 222 aa, synthetic construct
  source 1..222: note = switchable chimeric antigen receptor
EFKPLPEVTDEYGGGGSEFKPLPEVTDEYESKYGPPCPPCPMFWVLVVVGGVLACYSLLVTVAFIIFWVRSKRSRGGHSDYMNMTPRRPGPTRKHYQPYAPPRDFAAYRSRVKFSRSADAPAYQQGQNQLYNELNLGRREEYDVLDKRRGRDPEMGGKPRRKNPQEGLYNELQKDKMAEAYSEIGMKGERRRGKGHDGLYQGLSTATKDTYDALHMQALPPR

SEQ ID NO: 96 - protein, 219 aa, synthetic construct
  source 1..219: note = switchable chimeric antigen receptor
EFKPLPEVTDEYGGGGSEFKPLPEVTDEYESKYGPPCPPCPDIYIWAPLAGTCGVLLLSLVITLYCRSKRSRGGHSDYMNMTPRRPGPTRKHYQPYAPPRDFAAYRSRVKFSRSADAPAYQQGQNQLYNELNLGRREEYDVLDKRRGRDPEMGGKPRRKNPQEGLYNELQKDKMAEAYSEIGMKGERRRGKGHDGLYQGLSTATKDTYDALHMQALPPR

SEQ ID NO: 97 - protein, 223 aa, synthetic construct
  source 1..223: note = switchable chimeric antigen receptor
EFKPLPEVTDEYGGGGSEFKPLPEVTDEYESKYGPPCPPCPMFWVLVVVGGVLACYSLLVTVAFIIFWVKRGRKKLLYIFKQPFMRPVQTTQEEDGCSCRFPEEEEGGCELRVKFSRSADAPAYQQGQNQLYNELNLGRREEYDVLDKRRGRDPEMGGKPRRKNPQEGLYNELQKDKMAEAYSEIGMKGERRRGKGHDGLYQGLSTATKDTYDALHMQALPPR

SEQ ID NO: 98 - protein, 223 aa, synthetic construct
  source 1..223: note = switchable chimeric antigen receptor
EFKPLPEVTDEYGGGGSEFKPLPEVTDEYESKYGPPCPPCPMFWVLVVVGGVLACYSLLVTVAFIIFWVKRGRKKGGYIFKQPFMRPVQTTQEEDGCSCRFPEEEEGGCELRVKFSRSADAPAYQQGQNQLYNELNLGRREEYDVLDKRRGRDPEMGGKPRRKNPQEGLYNELQKDKMAEAYSEIGMKGERRRGKGHDGLYQGLSTATKDTYDALHMQALPPR

SEQ ID NO: 99 - protein, 214 aa, synthetic construct
  source 1..214: note = switchable chimeric antigen receptor
EFKPLPEVTDEYAAAGGSGGSESKYGPPCPPCPMFWVLVVVGGVLACYSLLVTVAFIIFWVRSKRSRLLHSDYMNMTPRRPGPTRKHYQPYAPPRDFAAYRSRVKFSRSADAPAYQQGQNQLYNELNLGRREEYDVLDKRRGRDPEMGGKPRRKNPQEGLYNELQKDKMAEAYSEIGMKGERRRGKGHDGLYQGLSTATKDTYDALHMQALPPR

SEQ ID NO: 100 - protein, 214 aa, synthetic construct
  source 1..214: note = switchable chimeric antigen receptor
EFKPLPEVTDEYAAAGGSGGSESKYGPPCPPCPMFWVLVVVGGVLACYSLLVTVAFIIFWVRSKRSRGGHSDYMNMTPRRPGPTRKHYQPYAPPRDFAAYRSRVKFSRSADAPAYQQGQNQLYNELNLGRREEYDVLDKRRGRDPEMGGKPRRKNPQEGLYNELQKDKMAEAYSEIGMKGERRRGKGHDGLYQGLSTATKDTYDALHMQALPPR

SEQ ID NO: 101 - protein, 211 aa, synthetic construct
  source 1..211: note = switchable chimeric antigen receptor
EFKPLPEVTDEYAAAGGSGGSESKYGPPCPPCPDIYIWAPLAGTCGVLLLSLVITLYCRSKRSRGGHSDYMNMTPRRPGPTRKHYQPYAPPRDFAAYRSRVKFSRSADAPAYQQGQNQLYNELNLGRREEYDVLDKRRGRDPEMGGKPRRKNPQEGLYNELQKDKMAEAYSEIGMKGERRRGKGHDGLYQGLSTATKDTYDALHMQALPPR

SEQ ID NO: 102 - protein, 215 aa, synthetic construct
  source 1..215: note = switchable chimeric antigen receptor
EFKPLPEVTDEYAAAGGSGGSESKYGPPCPPCPMFWVLVVVGGVLACYSLLVTVAFIIFWVKRGRKKLLYIFKQPFMRPVQTTQEEDGCSCRFPEEEEGGCELRVKFSRSADAPAYQQGQNQLYNELNLGRREEYDVLDKRRGRDPEMGGKPRRKNPQEGLYNELQKDKMAEAYSEIGMKGERRRGKGHDGLYQGLSTATKDTYDALHMQALPPR

SEQ ID NO: 103 - protein, 215 aa, synthetic construct
  source 1..215: note = switchable chimeric antigen receptor
EFKPLPEVTDEYAAAGGSGGSESKYGPPCPPCPMFWVLVVVGGVLACYSLLVTVAFIIFWVKRGRKKGGYIFKQPFMRPVQTTQEEDGCSCRFPEEEEGGCELRVKFSRSADAPAYQQGQNQLYNELNLGRREEYDVLDKRRGRDPEMGGKPRRKNPQEGLYNELQKDKMAEAYSEIGMKGERRRGKGHDGLYQGLSTATKDTYDALHMQALPPR

SEQ ID NO: 104 - protein, 246 aa, synthetic construct
  source 1..246: note = switchable chimeric antigen receptor
EFKPLPEVTDEYGGGGSEFKPLPEVTDEYIEVMYPPPYLDNEKSNGTIIHVKGKHLCPSPLFPGPSKPDIYIWAPLAGTCGVLLLSLVITLYCRSKRSRGGHSDYMNMTPRRPGPTRKHYQPYAPPRDFAAYRSRVKFSRSADAPAYQQGQNQLYNELNLGRREEYDVLDKRRGRDPEMGGKPRRKNPQEGLYNELQKDKMAEAYSEIGMKGERRRGKGHDGLYQGLSTATKDTYDALHMQALPPR

SEQ ID NO: 105 - protein, 205 aa, synthetic construct
  source 1..205: note = switchable chimeric antigen receptor
EFKPLPEVTDEYESKYGPPCPPCPMFWVLVVVGGVLACYSLLVTVAFIIFWVRSKRSRGGHSDYMNMTPRRPGPTRKHYQPYAPPRDFAAYRSRVKFSRSADAPAYQQGQNQLYNELNLGRREEYDVLDKRRGRDPEMGGKPRRKNPQEGLYNELQKDKMAEAYSEIGMKGERRRGKGHDGLYQGLSTATKDTYDALHMQALPPR

SEQ ID NO: 106 - protein, 206 aa, synthetic construct
  source 1..206: note = switchable chimeric antigen receptor
EFKPLPEVTDEYESKYGPPCPPCPMFWVLVVVGGVLACYSLLVTVAFIIFWVKRGRKKGGYIFKQPFMRPVQTTQEEDGCSCRFPEEEEGGCELRVKFSRSADAPAYQQGQNQLYNELNLGRREEYDVLDKRRGRDPEMGGKPRRKNPQEGLYNELQKDKMAEAYSEIGMKGERRRGKGHDGLYQGLSTATKDTYDALHMQALPPR

SEQ ID NO: 107 - protein, 212 aa, synthetic construct; identical to SEQ ID NO: 88
  source 1..212: note = switchable chimeric antigen receptor

SEQ ID NO: 108 - DNA, 660 bp, synthetic construct
  source 1..660: mol_type = other DNA; note = nucleic acid encoding switchable chimeric antigen receptor
gagttcaagcctctgcctgaagtgaccgatgagtatgccgctgctggtggatctggcggcagcgagtctaagtacggacctccttgtcctccatgtcctaccagaggcctggacttcgcctgcgacatctatatctgggcccctctggctggcacatgtggcgttttgctgctgagcctggtcatcaccctgtactgcaagcggggcagaaagaagctgctgtacatcttcaagcagcccttcatgcggcccgtgcagaccacacaagaggaagatggctgctcctgcagattccccgaggaagaagaaggcggctgcgagctgagagtgaagttcagcagatccgccgacgctcccgcctataagcagggacagaaccagctgtacaacgagctgaacctggggagaagagaagagtacgacgtgctggacaagcggagaggcagagatcctgagatgggcggcaagcccagacggaagaatcctcaagagggcctgtataatgagctgcagaaagacaagatggccgaggcctacagcgagatcggaatgaagggcgagcgcagaagaggcaagggacacgatggactgtaccagggcctgagcaccgccaccaaggatacctatgatgccctgcacatgcaggccctgcctccaaga

SEQ ID NO: 109 - DNA, 732 bp, synthetic construct
  source 1..732: mol_type = other DNA; note = nucleic acid encoding switchable chimeric antigen receptor
gagttcaagcctctgcctgaagtgaccgatgagtatgccgctgctggtggatctggcggcagcacaacaacaccagctcctagaccacctacaccagcacctaccattgccagccagcctctgtctctgaggccagaggcatgtagacctgctgctggcggagccgtgcatacaagaggactggatttcgcctgcgacatctacatctgggcccctctggctggaacatgtggcgttctgctgctgagcctggtcatcaccctgtactgcaagcggggcagaaagaagctgctgtacatcttcaagcagcccttcatgcggcccgtgcagaccacacaagaggaagatggctgctcctgcagattccccgaggaagaagaaggcggctgcgagctgagagtgaagttcagcagatccgccgacgctcccgcctataagcagggacagaaccagctgtacaacgagctgaacctggggagaagagaagagtacgacgtgctggacaagcggagaggcagagatcctgagatgggcggcaagcccagacggaagaatcctcaagagggcctgtataatgagctgcagaaagacaagatggccgaggcctacagcgagatcggaatgaagggcgagcgcagaagaggcaagggacacgatggactgtaccagggcctgagcaccgccaccaaggatacctatgatgccctgcacatgcaggccctgcctccaaga

SEQ ID NO: 110 - DNA, 720 bp, synthetic construct
  source 1..720: mol_type = other DNA; note = nucleic acid encoding switchable chimeric antigen receptor
gagttcaagcctctgcctgaagtgaccgatgagtatgccgctgctggtggatctggcggcagcatcgaagtgatgtaccctccaccttacctggacaacgagaagtccaacggcaccatcatccacgtgaagggcaagcacctgtgtccttctccactgttccccggacctagcaagcctttctgggtgctcgttgttgttggcggcgtgctggcctgttacagcctgctggttaccgtggccttcatcatcttttgggtccgaagcaagcggagccggctgctgcacagcgactacatgaacatgacccctagacggcccggaccaaccagaaagcactaccagccttacgctcctcctagagacttcgccgcctaccggtccagagtgaagttcagcagatccgccgatgctcccgcctatcagcagggacagaaccagctgtacaacgagctgaacctggggagaagagaagagtacgacgtgctggacaagcggagaggcagagatcctgagatgggcggcaagcccagacggaagaatcctcaagagggcctgtataatgagctgcagaaagacaagatggccgaggcctacagcgagatcggaatgaagggcgagcgcagaagaggcaagggacacgatggactgtaccagggactgagcaccgccaccaaggatacctatgacgccctgcacatgcaggccctgcctccaaga

SEQ ID NO: 111 - DNA, 771 bp, synthetic construct
  source 1..771: mol_type = other DNA; note = nucleic acid encoding switchable chimeric antigen receptor
gagttcaagcctctgcctgaagtgaccgatgagtatgccgctgctggtggaagcggcggctctttcgttcctgtgttcctgcctgccaagcctaccaccacaccagctcctagacctccaactcctgctcctaccattgccagccagcctctgtctctgaggccagaggcatgtagacctgctgctggcggagccgtgcatacaagaggactggatttcgcctgcgacatctacatctgggcccctctggctggaacatgtggcgttctgctgctgagcctggtcatcaccctgtactgcaaccaccggaacagaagcaagcggagcagactgctgcacagcgactacatgaacatgacccctagacggcccggacctaccagaaagcactaccagccttacgctcctcctagagacttcgccgcctaccggtccagagtgaagttcagcagatccgccgatgctcccgcctatcagcagggacagaaccagctgtacaacgagctgaacctggggagaagagaagagtacgacgtgctggacaagcggagaggcagagatcctgagatgggcggcaagcccagacggaagaatcctcaagagggcctgtataatgagctgcagaaagacaagatggccgaggcctacagcgagatcggaatgaagggcgagcgcagaagaggcaagggacacgatggactgtaccagggcctgagcaccgccaccaaggatacctatgatgccctgcacatgcaggccctgcctccaaga

SEQ ID NO: 112 - DNA, 717 bp, synthetic construct
  source 1..717: mol_type = other DNA; note = nucleic acid encoding switchable chimeric antigen receptor
gagttcaagcctctgcctgaagtgaccgacgagtatggcggaagcggaggatctggcggatctaagccactgccagaagtcacagacgaatacgccgctgcaggcggttcaggcggatccgagtctaagtacggacctccttgtcctccatgtcctaccagaggcctggacttcgcctgcgacatctatatctgggcccctctggctggcacatgtggcgttttgctgctgagcctggtcatcaccctgtactgcaagcggggcagaaagaagctgctgtacatcttcaagcagcccttcatgcggcccgtgcagaccacacaagaggaagatggctgctcctgcagattccccgaggaagaagaaggcggctgcgagctgagagtgaagttcagcagatccgctgacgcccctgcctacaagcagggacagaaccagctgtacaacgagctgaacctggggagaagagaagagtacgacgtgctggacaagcggagaggcagagatcctgagatgggcggcaagcccagacggaagaatcctcaagagggcctgtataatgagctgcagaaagacaagatggccgaggcctacagcgagatcggaatgaagggcgagcgcagaagaggcaagggacacgatggactgtaccagggcctgagcaccgccaccaaggatacctatgatgccctgcacatgcaggccctgcctccaaga

SEQ ID NO: 113 - protein, 774 aa, synthetic construct
  source 1..774: note = nucleic acid encoding switchable chimeric antigen receptor
GAGTTCAAGCCTCTGCCTGAAGTGACCGACGAGTATGGCGGAAGCGGAGGATCTGGCGGATCTAAGCCACTGCCAGAAGTCACAGACGAATACGGCGGTTCAGGTGGCAGCGGAGGCTCTAAACCTCTTCCAGAAGTTACTGACGAGTACGCCGCTGCAGGCGGTTCTGGCGGCTCTGAGTCTAAGTACGGACCTCCTTGTCCTCCATGTCCTACCAGAGGCCTGGACTTCGCCTGCGACATCTATATCTGGGCCCCTCTGGCTGGCACATGTGGCGTTTTGCTGCTGAGCCTGGTCATCACCCTGTACTGCAAGCGGGGCAGAAAGAAGCTGCTGTACATCTTCAAGCAGCCCTTCATGCGGCCCGTGCAGACCACACAAGAGGAAGATGGCTGCTCCTGCAGATTCCCCGAGGAAGAAGAAGGCGGCTGCGAGCTGAGAGTGAAGTTCAGCAGATCCGCTGACGCCCCTGCCTACAAGCAGGGACAGAACCAGCTGTACAACGAGCTGAACCTGGGGAGAAGAGAAGAGTACGACGTGCTGGACAAGCGGAGAGGCAGAGATCCTGAGATGGGCGGCAAGCCCAGACGGAAGAATCCTCAAGAGGGCCTGTATAATGAGCTGCAGAAAGACAAGATGGCCGAGGCCTACAGCGAGATCGGAATGAAGGGCGAGCGCAGAAGAGGCAAGGGACACGATGGACTGTACCAGGGCCTGAGCACCGCCACCAAGGATACCTATGATGCCCTGCACATGCAGGCCCTTCCACCTCGC

SEQ ID NO: 114 - DNA, 1041 bp, synthetic construct
  source 1..1041: mol_type = other DNA; note = nucleic acid encoding switchable chimeric antigen receptor
gagttcaagcctctgcctgaagtgaccgatgagtacgccgctgctggacctggtggcggaggatctaagattctggtcaagcagagccccatgctggtggcctacgacaacgccgtgaatctgagctgcaagtacagctacaacctgttcagcagagagttccgggccagcctgcacaaaggactggattctgctgtggaagtgtgcgtggtgtacggcaactacagccagcagctgcaggtctacagcaagaccggcttcaactgcgacggcaagctgggcaatgagagcgtgaccttctacctgcaaaacctgtacgtgaaccagaccgatatctacttctgcaagatcgaagtgatggcccctcctcctgctctggacaacgagaagtccaacggcaccatcatccacgtgaagggcaagcacctgtgtccttctccactgttccccggacctagcaagcctttctgggtgctcgttgttgttggcggcgtgctggcctgttatagcctgctggttaccgtggccttcatcatcttttgggtccgaagcaggcggagcagaggcggccacagcgactacatgaacatgacccctagacggcccggaccaaccagaaagcactaccagccttacgctcctcctagagacttcgccgcctacagatctggcggaggtggaagcggaggcggagcttcaggcggtggcggatcttttagcagatccgccgatgctcctgcctaccagcagggacagaaccagctgtacaacgagctgaacctggggagaagagaagagtacgatgtgctggacaggcggagaggcagagatcctgaaatgggcggcagacccagacggcggaatcctcaagagggcctgtataatgagctgcagcgcgacagaatggccgaggcctattctgagatcggcatgagaggcgagcggagaagaggtagaggacacgatggcctgtaccagggcctgagcacagccaccagagatacttatggcgccctgcacatgcaggccctgcctccaaga

SEQ ID NO: 115 - DNA, 1047 bp, synthetic construct
  source 1..1047: mol_type = other DNA; note = nucleic acid encoding switchable chimeric antigen receptor
gagttcagcaagcctctgcctgaagtgaccgacgagtacaagaatgccgccgctggtggatctggcggctctaagattctggtcaagcagagccctatgctggtggcctacgacaacgccgtgaacctgagctgcaagtacagctacaacctgttcagcagagagttccgggccagcctgcacaaaggactggattctgctgtggaagtgtgcgtggtgtacggcaactacagccagcagctgcaggtctacagcaagaccggcttcaactgcgacggcaagctgggcaatgagagcgtgaccttctacctgcaaaacctgtacgtgaaccagaccgatatctacttctgcaagatcgaagtgatggcccctcctcctgctctggacaacgagaagtccaacggcaccatcatccacgtgaagggcaagcacctgtgtccttctccactgttccccggacctagcaagcctttctgggtgctcgttgttgttggcggcgtgctggcctgttatagcctgctggttaccgtggccttcatcatcttttgggtccgaagcaagcggagcagaggcggccacagcgactacatgaacatgacccctagacggcccggaccaaccagaaagcactaccagccttacgctcctcctagagacttcgccgcctatagaagcggaggcggaggttctggtggcggtgcttctggcggcggaggaagcttttccagatctgccgatgctcccgcctatcagcagggccagaaccagctgtacaacgagctgaacctggggagaagagaagagtacgacgtgctggacaagcggagaggcagagatcctgagatgggcggcaagcccagacggaagaatcctcaagagggcctgtacaatgaactgcagaaagacaagatggccgaggcctacagcgagatcggaatgaagggcgagcgcagaagaggcaagggacacgatggactgtaccagggcctgagcacagccaccaaggatacttatggcgccctgcacatgcaggccctgcctccaaga

SEQ ID NO: 116 - DNA, 609 bp, synthetic construct
  source 1..609: mol_type = other DNA; note = nucleic acid encoding switchable chimeric antigen receptor
gagttcaagcctctgcctgaagtgaccgacgagtacgagtctaagtacggccctccttgtcctccatgtcctgacatctacatctgggcccctctggccggaacatgtggtgttctgctgctgagcctggtcatcaccctgtactgcaagcggggcagaaagaagctgctgtacatcttcaagcagcccttcatgcggcccgtgcagaccacacaagaggaagatggctgctcctgcagattccccgaggaagaagaaggcggctgcgagctgagagtgaagttcagcagatccgccgacgctcctgcctatcagcagggacagaaccagctgtacaacgagctgaacctggggagaagagaagagtacgacgtgctggacaagcggagaggcagagatcctgagatgggcggcaagcccagacggaagaatcctcaagagggcctgtataatgagctgcagaaagacaagatggccgaggcctacagcgagatcggaatgaagggcgagcgcagaagaggcaagggacacgatggactgtaccagggcctgagcaccgccaccaaggatacctatgatgccctgcacatgcaggccctgcctccaaga

SEQ ID NO: 117 - DNA, 618 bp, synthetic construct
  source 1..618: mol_type = other DNA; note = nucleic acid encoding switchable chimeric antigen receptor
gagttcaagcctctgcctgaagtgaccgacgagtatgccgccgctgagtctaagtacggccctccttgtcctccatgtcctgacatctacatctgggcccctctggccggaacatgtggtgttctgctgctgagcctggtcatcaccctgtactgcaagcggggcagaaagaagctgctgtacatcttcaagcagcccttcatgcggcccgtgcagaccacacaagaggaagatggctgctcctgcagattccccgaggaagaagaaggcggctgcgagctgagagtgaagttcagcagatccgccgacgctcctgcctatcagcagggacagaaccagctgtacaacgagctgaacctggggagaagagaagagtacgacgtgctggacaagcggagaggcagagatcctgagatgggcggcaagcccagacggaagaatcctcaagagggcctgtataatgagctgcagaaagacaagatggccgaggcctacagcgagatcggaatgaagggcgagcgcagaagaggcaagggacacgatggactgtaccagggcctgagcaccgccaccaaggatacctatgatgccctgcacatgcaggccctgcctccaaga

SEQ ID NO: 118 - DNA, 636 bp, synthetic construct
  source 1..636: mol_type = other DNA; note = nucleic acid encoding switchable chimeric antigen receptor
gagttcaagcctctgcctgaagtgaccgatgagtatgccgctgctggtggatctggcggcagcgagtctaagtacggacctccttgtcctccatgtcctgacatctacatctgggcccctctggccggaacatgtggtgttctgctgctgagcctggtcatcaccctgtactgcaagcggggcagaaagaagctgctgtacatcttcaagcagcccttcatgcggcccgtgcagaccacacaagaggaagatggctgctcctgcagattccccgaggaagaagaaggcggctgcgagctgagagtgaagttcagcagatccgccgacgctcctgcctatcagcagggacagaaccagctgtacaacgagctgaacctggggagaagagaagagtacgacgtgctggacaagcggagaggcagagatcctgagatgggcggcaagcccagacggaagaatcctcaagagggcctgtataatgagctgcagaaagacaagatggccgaggcctacagcgagatcggaatgaagggcgagcgcagaagaggcaagggacacgatggactgtaccagggcctgagcaccgccaccaaggatacctatgatgccctgcacatgcaggccctgcctccaaga

SEQ ID NO: 119 - DNA, 621 bp, synthetic construct
  source 1..621: mol_type = other DNA; note = nucleic acid encoding switchable chimeric antigen receptor
agcaagcccctgcctgaagtgaccgacgagtacaagaatgccgccgctgagtctaagtacggccctccttgtcctccatgtcctgacatctatatctgggcccctctggccggaacatgtggcgttttgctgctgagcctggtcatcaccctgtactgcaagcggggcagaaagaagctgctgtacatcttcaagcagcccttcatgcggcccgtgcagaccacacaagaggaagatggctgctcctgcagattccccgaggaagaagaaggcggctgcgagctgagagtgaagttcagcagatccgccgacgctcctgcctatcagcagggacagaaccagctgtacaacgagctgaacctggggagaagagaagagtacgacgtgctggacaagcggagaggcagagatcctgagatgggcggcaagcccagacggaagaatcctcaagagggcctgtataatgagctgcagaaagacaagatggccgaggcctacagcgagatcggaatgaagggcgagcgcagaagaggcaagggacacgatggactgtaccagggcctgagcaccgccaccaaggatacctatgatgccctgcacatgcaggccctgcctccaaga

SEQ ID NO: 120 - DNA, 1119 bp, synthetic construct
  source 1..1119: mol_type = other DNA; note = nucleic acid encoding switchable chimeric antigen receptor
gagaacggcgacaacgagaaaatggccgctctggaagccaagatctgccaccagatcgagtactacttcggcgacttcaacctgcctcgggacaagttcctgaaagagcagatcaagctggacgaaggctgggtgcccctggaaatcatgatcaagttcaaccggctgaacaggctgaccaccgacttcaatgtgatcgtggaagccctgagcaagagcaaggccgagctgatggaaatcagcgaggacaagaccaagatccggcggagcccttctaagcccctgcctgaagtgaccgacgagtacaagaacgacgtgaagaaccgcagcgtgtacatcaagggcttccccaccgatgccacactggacgacatcaaagagtggcttgaggacaaaggccaggtgctgaacatccagatgcggcggacactgcacaaggccttcaagggcagcatcttcgtggtgttcgacagcatcgagagcgccaagaaattcgtggaaacccctggccagaagtacaaagagacagacctgctgatcctgttcgagtctaagtacggccctccttgtcctccatgtcctgacatctacatctgggcccctctggccggaacatgtggtgttctgctgctgagcctggtcatcaccctgtactgcaagcggggcagaaagaagctgctgtacatcttcaagcagcccttcatgcggcccgtgcagaccacacaagaggaagatggctgctcctgcagattccccgaggaagaagaaggcggctgcgagctgagagtgaagttcagcagatccgccgacgctcctgcctatcagcagggacagaaccagctgtacaacgagctgaacctggggagaagagaagagtacgacgtgctggacaagcggagaggcagagatcctgagatgggcggcaagcccagacggaagaatcctcaagagggcctgtataatgagctgcagaaagacaagatggccgaggcctacagcgagatcggaatgaagggcgagcgcagaagaggcaagggacacgatggactgtaccagggcctgagcaccgccaccaaggatacctatgatgccctgcacatgcaggccctgcctccaaga

SEQ ID NO: 121 - DNA, 661 bp, synthetic construct
  source 1..661: mol_type = other DNA; note = nucleic acid encoding switchable chimeric antigen receptor
gagttcaagcctctgcctgaagtgaccgacgagtatggcggcggaggcagcgagtttaaacccctgccagaagtcacagacgaatacgagtctaagtacggccctccttgtcctccatgtcctgacatctacatctgggcccctctggccggaacatgtggtgttctgctgctgagcctggtcatcaccctgtactgcaagcggggcagaaagaagctgctgtacatcttcaagcagcccttcatgcggcccgtgcagaccacacaagaggaagatggctgctcctgcagattccccgaggaagaagaaggcggctgcgagctgagagtgaagttcagcagatccgccgacgctcctgcctatcagcagggacagaaccagctgtacaacgagctgaacctggggagaagagaagagtacgacgtgctggacaagcggagaggcagagatcctgagatgggcggcaagcccagacggaagaatcctcaagagggcctgtataatgagctgcagaaagacaagatggccgaggcctacagcgagatcggaatgaagggcgagcgcagaagaggcaagggacacgatggactgtaccagggcctgagcaccgccaccaaggatacctatgatgccctgcacatgcaggccctgcctccaagag

SEQ ID NO: 122 - DNA, 624 bp, synthetic construct
  source 1..624: mol_type = other DNA; note = nucleic acid encoding switchable chimeric antigen receptor
gagttcaagcctctgcctgaagtgaccgacgagtatgccgccgctgagtctaagtacggccctccttgtcctccatgtcctatgttctgggtgctcgtggttgttggcggagtgctggcctgttacagcctgctggttaccgtggccttcatcatcttttgggtccgaagcaagcggagccggctgctgcacagcgactacatgaacatgacccctagacggcccggacctaccagaaagcactaccagccttacgctcctcctagagacttcgccgcctaccggtccagagtgaagttcagcagatccgccgatgctcccgcctatcagcagggacagaaccagctgtacaacgagctgaacctggggagaagagaagagtacgacgtgctggacaagcggagaggcagagatcctgagatgggcggcaagcccagacggaagaatcctcaagagggcctgtataatgagctgcagaaagacaagatggccgaggcctacagcgagatcggaatgaagggcgagcgcagaagaggcaagggacacgatggactgtaccagggactgagcaccgccaccaaggatacctatgacgccctgcacatgcaggccctgcctccaaga

SEQ ID NO: 123 - DNA, 627 bp, synthetic construct
  source 1..627: mol_type = other DNA; note = nucleic acid encoding switchable chimeric antigen receptor
gagttcaagcctctgcctgaagtgaccgacgagtatgccgccgctgagtctaagtacggccctccttgtcctccatgtcctatgttctgggtgctcgtggttgttggcggagtgctggcctgttacagcctgctggttaccgtggccttcatcatcttttgggtcaagcggggcagaaagaagctgctgtacatcttcaagcagcccttcatgcggcccgtgcagaccacacaagaggaagatggctgctcctgcagattccccgaggaagaagaaggcggctgcgagctgagagtgaagttcagcagatccgccgacgctcctgcctatcagcagggacagaaccagctgtacaacgagctgaacctggggagaagagaagagtacgacgtgctggacaagcggagaggcagagatcctgagatgggcggcaagcccagacggaagaatcctcaagagggcctgtataatgagctgcagaaagacaagatggccgaggcctacagcgagatcggaatgaagggcgagcgcagaagaggcaagggacacgatggactgtaccagggactgagcaccgccaccaaggatacctatgacgccctgcacatgcaggccctgcctccaaga

SEQ ID NO: 124 - DNA, 666 bp, synthetic construct
  source 1..666: mol_type = other DNA; note = nucleic acid encoding switchable chimeric antigen receptor
gagttcaagcctctgcctgaagtgaccgacgagtatggcggcggaggcagcgagtttaaacccctgccagaagtcacagacgaatacgagtctaagtacggccctccttgtcctccatgtcctatgttctgggtgctcgtggttgttggcggagtgctggcctgttacagcctgctggttaccgtggccttcatcatcttttgggtccgaagcaagcggagccggctgctgcacagcgactacatgaacatgacccctagacggcccggacctaccagaaagcactaccagccttacgctcctcctagagacttcgccgcctaccggtccagagtgaagttcagcagatccgccgatgctcccgcctatcagcagggacagaaccagctgtacaacgagctgaacctggggagaagagaagagtacgacgtgctggacaagcggagaggcagagatcctgagatgggcggcaagcccagacggaagaatcctcaagagggcctgtataatgagctgcagaaagacaagatggccgaggcctacagcgagatcggaatgaagggcgagcgcagaagaggcaagggacacgatggactgtaccagggactgagcaccgccaccaaggatacctatgacgccctgcacatgcaggccctgcctccaaga

SEQ ID NO: 125 - DNA, 666 bp, synthetic construct
  source 1..666: mol_type = other DNA; note = nucleic acid encoding switchable chimeric antigen receptor
gagttcaagcctctgcctgaagtgaccgacgagtatggcggcggaggcagcgagtttaaacccctgccagaagtcacagacgaatacgagtctaagtacggccctccttgtcctccatgtcctatgttctgggtgctcgtggttgttggcggagtgctggcctgttacagcctgctggttaccgtggccttcatcatcttttgggtccgaagcaagcggagcagaggcggccacagcgactacatgaacatgacccctagacggcccggacctaccagaaagcactaccagccttacgctcctcctagagacttcgccgcctaccggtccagagtgaagttcagcagatccgccgatgctcccgcctatcagcagggacagaaccagctgtacaacgagctgaacctggggagaagagaagagtacgacgtgctggacaagcggagaggcagagatcctgagatgggcggcaagcccagacggaagaatcctcaagagggcctgtataatgagctgcagaaagacaagatggccgaggcctacagcgagatcggaatgaagggcgagcgcagaagaggcaagggacacgatggactgtaccagggactgagcaccgccaccaaggatacctatgacgccctgcacatgcaggccctgcctccaaga

SEQ ID NO: 126 - DNA, 657 bp, synthetic construct
  source 1..657: mol_type = other DNA; note = nucleic acid encoding switchable chimeric antigen receptor
gagttcaagcctctgcctgaagtgaccgacgagtatggcggcggaggcagcgagtttaaacccctgccagaagtcacagacgaatacgagtctaagtacggccctccttgtcctccatgtcctgacatctacatctgggcccctctggccggaacatgtggtgttctgctgctgagcctggtcatcaccctgtactgcagaagcaagagaagcagaggcggccacagcgactacatgaacatgacccctagacggcccggacctaccagaaagcactaccagccttacgctcctcctagagacttcgccgcctaccggtccagagtgaagttcagcagatccgccgatgctcccgcctatcagcagggacagaaccagctgtacaacgagctgaacctggggagaagagaagagtacgacgtgctggacaagcggagaggcagagatcctgagatgggcggcaagcccagacggaagaatcctcaagagggcctgtataatgagctgcagaaagacaagatggccgaggcctacagcgagatcggaatgaagggcgaacgcagaagaggcaagggccacgatggactgtatcagggcctgagcaccgccaccaaggatacctatgatgccctgcacatgcaggccctgcctccaaga

SEQ ID NO: 127 - DNA, 669 bp, synthetic construct
  source 1..669: mol_type = other DNA; note = nucleic acid encoding switchable chimeric antigen receptor
gagttcaagcctctgcctgaagtgaccgacgagtatggcggcggaggcagcgagtttaaacccctgccagaagtcacagacgaatacgagtctaagtacggccctccttgtcctccatgtcctatgttctgggtgctcgtggttgttggcggagtgctggcctgttacagcctgctggttaccgtggccttcatcatcttttgggtcaagcggggcagaaagaagctgctgtacatcttcaagcagcccttcatgcggcccgtgcagaccacacaagaggaagatggctgctcctgcagattccccgaggaagaagaaggcggctgcgagctgagagtgaagttcagcagatccgccgacgctcctgcctatcagcagggacagaaccagctgtacaacgagctgaacctggggagaagagaagagtacgacgtgctggacaagcggagaggcagagatcctgagatgggcggcaagcccagacggaagaatcctcaagagggcctgtataatgagctgcagaaagacaagatggccgaggcctacagcgagatcggaatgaagggcgagcgcagaagaggcaagggacacgatggactgtaccagggactgagcaccgccaccaaggatacctatgacgccctgcacatgcaggccctgcctccaaga

SEQ ID NO: 128 - DNA, 669 bp, synthetic construct
  source 1..669: mol_type = other DNA; note = nucleic acid encoding switchable chimeric antigen receptor
gagttcaagcctctgcctgaagtgaccgacgagtatggcggcggaggcagcgagtttaaacccctgccagaagtcacagacgaatacgagtctaagtacggccctccttgtcctccatgtcctatgttctgggtgctcgtggttgttggcggagtgctggcctgttacagcctgctggttaccgtggccttcatcatcttttgggtcaagcggggcagaaagaaaggcggctacatcttcaagcagcccttcatgaggcccgtgcagaccacacaagaggaagatggctgctcctgcagattccccgaggaagaagaaggcggctgcgagctgagagtgaagttcagcagatccgccgacgctcctgcctatcagcagggacagaaccagctgtacaacgagctgaacctggggagaagagaagagtacgacgtgctggacaagcggagaggcagagatcctgagatgggcggcaagcccagacggaagaatcctcaagagggcctgtataatgagctgcagaaagacaagatggccgaggcctacagcgagatcggaatgaagggcgagcgcagaagaggcaagggacacgatggactgtaccagggactgagcaccgccaccaaggatacctatgacgccctgcacatgcaggccctgcctccaaga

SEQ ID NO: 129 - DNA, 642 bp, synthetic construct
  source 1..642: mol_type = other DNA; note = nucleic acid encoding switchable chimeric antigen receptor
gagttcaagcctctgcctgaagtgaccgatgagtatgccgctgctggtggatctggcggcagcgagtctaagtacggacctccttgtcctccatgtcctatgttctgggtgctcgtggttgttggcggagtgctggcctgttacagcctgctggttaccgtggccttcatcatcttttgggtccgaagcaagcggagccggctgctgcacagcgactacatgaacatgacccctagacggcccggacctaccagaaagcactaccagccttacgctcctcctagagacttcgccgcctaccggtccagagtgaagttcagcagatccgccgatgctcccgcctatcagcagggacagaaccagctgtacaacgagctgaacctggggagaagagaagagtacgacgtgctggacaagcggagaggcagagatcctgagatgggcggcaagcccagacggaagaatcctcaagagggcctgtataatgagctgcagaaagacaagatggccgaggcctacagcgagatcggaatgaagggcgagcgcagaagaggcaagggacacgatggactgtaccagggactgagcaccgccaccaaggatacctatgacgccctgcacatgcaggccctgcctccaaga

SEQ ID NO: 130 - DNA, 642 bp, synthetic construct
  source 1..642: mol_type = other DNA; note = nucleic acid encoding switchable chimeric antigen receptor
gagttcaagcctctgcctgaagtgaccgatgagtatgccgctgctggtggatctggcggcagcgagtctaagtacggacctccttgtcctccatgtcctatgttctgggtgctcgtggttgttggcggagtgctggcctgttacagcctgctggttaccgtggccttcatcatcttttgggtccgaagcaagcggagcagaggcggccacagcgactacatgaacatgacccctagacggcccggacctaccagaaagcactaccagccttacgctcctcctagagacttcgccgcctaccggtccagagtgaagttcagcagatccgccgatgctcccgcctatcagcagggacagaaccagctgtacaacgagctgaacctggggagaagagaagagtacgacgtgctggacaagcggagaggcagagatcctgagatgggcggcaagcccagacggaagaatcctcaagagggcctgtataatgagctgcagaaagacaagatggccgaggcctacagcgagatcggaatgaagggcgagcgcagaagaggcaagggacacgatggactgtaccagggactgagcaccgccaccaaggatacctatgacgccctgcacatgcaggccctgcctccaaga

SEQ ID NO: 131 - DNA, 633 bp, synthetic construct
  source 1..633: mol_type = other DNA; note = nucleic acid encoding switchable chimeric antigen receptor
gagttcaagcctctgcctgaagtgaccgatgagtatgccgctgctggtggatctggcggcagcgagtctaagtacggacctccttgtcctccatgtcctgacatctacatctgggcccctctggccggaacatgtggtgttctgctgctgagcctggtcatcaccctgtactgcagaagcaagagaagcagaggcggccacagcgactacatgaacatgacccctagacggcccggacctaccagaaagcactaccagccttacgctcctcctagagacttcgccgcctaccggtccagagtgaagttcagcagatccgccgatgctcccgcctatcagcagggacagaaccagctgtacaacgagctgaacctggggagaagagaagagtacgacgtgctggacaagcggagaggcagagatcctgagatgggcggcaagcccagacggaagaatcctcaagagggcctgtataatgagctgcagaaagacaagatggccgaggcctacagcgagatcggaatgaagggcgaacgcagaagaggcaagggccacgatggactgtatcagggcctgagcaccgccaccaaggatacctatgatgccctgcacatgcaggccctgcctccaaga

SEQ ID NO: 132 - DNA, 645 bp, synthetic construct
  source 1..645: mol_type = other DNA; note = nucleic acid encoding switchable chimeric antigen receptor
gagttcaagcctctgcctgaagtgaccgatgagtatgccgctgctggtggatctggcggcagcgagtctaagtacggacctccttgtcctccatgtcctatgttctgggtgctcgtggttgttggcggagtgctggcctgttacagcctgctggttaccgtggccttcatcatcttttgggtcaagcggggcagaaagaagctgctgtacatcttcaagcagcccttcatgcggcccgtgcagaccacacaagaggaagatggctgctcctgcagattccccgaggaagaagaaggcggctgcgagctgagagtgaagttcagcagatccgccgacgctcctgcctatcagcagggacagaaccagctgtacaacgagctgaacctggggagaagagaagagtacgacgtgctggacaagcggagaggcagagatcctgagatgggcggcaagcccagacggaagaatcctcaagagggcctgtataatgagctgcagaaagacaagatggccgaggcctacagcgagatcggaatgaagggcgagcgcagaagaggcaagggacacgatggactgtaccagggactgagcaccgccaccaaggatacctatgacgccctgcacatgcaggccctgcctccaaga

SEQ ID NO: 133 - DNA, 645 bp, synthetic construct
  source 1..645: mol_type = other DNA; note = nucleic acid encoding switchable chimeric antigen receptor
gagttcaagcctctgcctgaagtgaccgatgagtatgccgctgctggtggctctggcggcagcgagtctaaatacggacctccttgtcctccatgtcctatgttctgggtgctcgtggttgttggcggagtgctggcctgttacagcctgctggttaccgtggccttcatcatcttttgggtcaagcggggcagaaagaaaggcggctacatcttcaagcagcccttcatgaggcccgtgcagaccacacaagaggaagatggctgctcctgcagattccccgaggaagaagaaggcggctgcgagctgagagtgaagttcagcagatccgccgacgctcctgcctatcagcagggacagaaccagctgtacaacgagctgaacctggggagaagagaagagtacgacgtgctggacaagcggagaggcagagatcctgagatgggcggcaagcccagacggaagaatcctcaagagggcctgtataatgagctgcagaaagacaagatggccgaggcctacagcgagatcggaatgaagggcgagcgcagaagaggcaagggacacgatggactgtaccagggactgagcaccgccaccaaggatacctatgacgccctgcacatgcaggccctgcctccaaga

SEQ ID NO: 134 - DNA, 738 bp, synthetic construct
  source 1..738: mol_type = other DNA; note = nucleic acid encoding switchable chimeric antigen receptor
gagtttaaaccactgcctgaggtgaccgatgagtacggcggcggcggcagcgagttcaagcccctgcctgaggtgactgatgagtatatcgaagtgatgtaccctcccccctatctggacaacgaaaaatctaacggcaccatcatccacgtcaaaggcaaacacctgtgcccatccccactgttccctggcccatctaagcccgacatctacatctgggcccctctggccggcacatgcggcgtgctgctgctcagcctggtgattacactgtactgccggtccaagagatccaggggcggccactctgactacatgaacatgacccccaggagacccggccccaccaggaaacactaccagccctacgcccccccccgggattttgccgcttaccgctccagggtgaagtttagcagatccgctgatgcccctgcctatcagcagggacagaaccagctgtacaacgagctgaacctggggagaagagaagagtacgatgtgctggacaagcggagaggcagagatcctgagatgggcggcaagcccagacggaagaatcctcaagagggcctgtacaatgaactgcagaaagacaagatggccgaggcctacagcgagatcggaatgaagggcgagcgcagaagaggcaagggacacgatggactgtaccagggcctgagcaccgccaccaaggatacctatgatgccctgcacatgcaggccctgcctccaaga

SEQ ID NO: 135 - DNA, 615 bp, synthetic construct
  source 1..615: mol_type = other DNA; note = nucleic acid encoding switchable chimeric antigen receptor
gagttcaagcctctgcctgaagtgaccgacgagtacgagtctaagtacggccctccttgtcctccatgtcctatgttctgggtgctcgtggttgttggcggagtgctggcctgttacagcctgctggttaccgtggccttcatcatcttttgggtccgaagcaagcggagcagaggcggccacagcgactacatgaacatgacccctagacggcccggacctaccagaaagcactaccagccttacgctcctcctagagacttcgccgcctaccggtccagagtgaagttcagcagatccgccgatgctcccgcctatcagcagggacagaaccagctgtacaacgagctgaacctggggagaagagaagagtacgacgtgctggacaagcggagaggcagagatcctgagatgggcggcaagcccagacggaagaatcctcaagagggcctgtataatgagctgcagaaagacaagatggccgaggcctacagcgagatcggaatgaagggcgagcgcagaagaggcaagggacacgatggactgtaccagggactgagcaccgccaccaaggatacctatgacgccctgcacatgcaggccctgcctccaaga

SEQ ID NO: 136 - DNA, 618 bp, synthetic construct
  source 1..618: mol_type = other DNA; note = nucleic acid encoding switchable chimeric antigen receptor
gagttcaagcctctgcctgaagtgaccgacgagtacgagtctaagtacggccctccttgtcctccatgtcctatgttctgggtgctcgtggttgttggcggagtgctggcctgttacagcctgctggttaccgtggccttcatcatcttttgggtcaagcggggcagaaagaaaggcggctacatcttcaagcagcccttcatgaggcccgtgcagaccacacaagaggaagatggctgctcctgcagattccccgaggaagaagaaggcggctgcgagctgagagtgaagttcagcagatccgccgacgctcctgcctatcagcagggacagaaccagctgtacaacgagctgaacctggggagaagagaagagtacgacgtgctggacaagcggagaggcagagatcctgagatgggcggcaagcccagacggaagaatcctcaagagggcctgtataatgagctgcagaaagacaagatggccgaggcctacagcgagatcggaatgaagggcgagcgcagaagaggcaagggacacgatggactgtaccagggactgagcaccgccaccaaggatacctatgacgccctgcacatgcaggccctgcctccaaga

SEQ ID NO: 137 - DNA, 636 bp, synthetic construct; identical to SEQ ID NO: 118
  source 1..636: mol_type = other DNA; note = nucleic acid encoding switchable chimeric antigen receptor